European Patent Application EP 4 613 776 A2, published September 10, 2025. Title: MULTIMERIC IL-15-BASED MOLECULES. Applicant: ALTOR BIOSCIENCE CORPORATION. Application EP. The sequence listing filed with the application follows.

SEQUENCE LISTING (58 sequences)

SEQ ID NO: 1 - DNA, 1125 bp, synthetic construct
  misc_feature 1..1125: note = Description of Artificial Sequence: Synthetic polynucleotide
  source 1..1125: mol_type = other DNA
atgaagtgggtgaccttcatcagcctgctgttcctgttctccagcgcctactccaacatccagatgacccagtcccctagctccgtgtccgcctccgtgggagatcgggtgaccatcacctgtagggcctcccaggacatctccaggtggctggcctggtaccagcagaagcccggcaaggcccccaagctgctgatctacgccgcctcctccctgcagtccggagtgcctagcaggttctccggctccggatccggcacagacttcgccctgaccatctcctccctgcagcccgaggacttcgccacctactactgccagcaggccgactccaggttctccatcaccttcggccagggcaccaggctggagatcaagaggggaggtggcggatccggaggtggaggttctggtggaggtgggagtgaggtgcagctggtgcagtccggaggaggactggtgcagcctggcggatccctgaggctgtcctgtgccgcttccggcttcaccttcagctcctactccatgaactgggtgaggcaggcccctggaaagggcctggagtgggtgtcctacatctccagctcctcctccaccatccagtacgccgactccgtgaagggcaggttcaccatctccagggacaacgccaagaactccctgtacctgcagatgaacagcctgagggacgaggacaccgccgtgtactactgcgccaggggcgactattactacggcatggacgtgtggggccagggaaccaccgtgaccgtgtcctccaactgggttaacgtaataagtgatttgaaaaaaattgaagatcttattcaatctatgcatattgatgctactttatatacggaaagtgatgttcaccccagttgcaaagtaacagcaatgaagtgctttctcttggagttacaagttatttcacttgagtccggagatgcaagtattcatgatacagtagaaaatctgatcatcctagcaaacgacagtttgtcttctaatgggaatgtaacagaatctggatgcaaagaatgtgaggaactggaggaaaaaaatattaaagaatttttgcagagttttgtacatattgtccaaatgttcatcaacacttcttaa

SEQ ID NO: 2 - protein, 374 aa, synthetic construct
  REGION 1..374: note = Description of Artificial Sequence: Synthetic polypeptide
MKWVTFISLLFLFSSAYSNIQMTQSPSSVSASVGDRVTITCRASQDISRWLAWYQQKPGKAPKLLIYAASSLQSGVPSRFSGSGSGTDFALTISSLQPEDFATYYCQQADSRFSITFGQGTRLEIKRGGGGSGGGGSGGGGSEVQLVQSGGGLVQPGGSLRLSCAASGFTFSSYSMNWVRQAPGKGLEWVSYISSSSSTIQYADSVKGRFTISRDNAKNSLYLQMNSLRDEDTAVYYCARGDYYYGMDVWGQGTTVTVSSNWVNVISDLKKIEDLIQSMHIDATLYTESDVHPSCKVTAMKCFLLELQVISLESGDASIHDTVENLIILANDSLSSNGNVTESGCKECEELEEKNIKEFLQSFVHIVQMFINTS

SEQ ID NO: 3 - DNA, 1674 bp, synthetic construct
  misc_feature 1..1674: note = Description of Artificial Sequence: Synthetic polynucleotide
  source 1..1674: mol_type = other DNA
atgaagtgggtgaccttcatcagcctgctgttcctgttctccagcgcctactccaacatccagatgacccagtcccctagctccgtgtccgcctccgtgggagatcgggtgaccatcacctgtagggcctcccaggacatctccaggtggctggcctggtaccagcagaagcccggcaaggcccccaagctgctgatctacgccgcctcctccctgcagtccggagtgcctagcaggttctccggctccggatccggcacagacttcgccctgaccatctcctccctgcagcccgaggacttcgccacctactactgccagcaggccgactccaggttctccatcaccttcggccagggcaccaggctggagatcaagaggggaggtggcggatccggaggtggaggttctggtggaggtgggagtgaggtgcagctggtgcagtccggaggaggactggtgcagcctggcggatccctgaggctgtcctgtgccgcttccggcttcaccttcagctcctactccatgaactgggtgaggcaggcccctggaaagggcctggagtgggtgtcctacatctccagctcctcctccaccatccagtacgccgactccgtgaagggcaggttcaccatctccagggacaacgccaagaactccctgtacctgcagatgaacagcctgagggacgaggacaccgccgtgtactactgcgccaggggcgactattactacggcatggacgtgtggggccagggaaccaccgtgaccgtgtcctccatcacgtgccctccccccatgtccgtggaacacgcagacatctgggtcaagagctacagcttgtactccagggagcggtacatttgtaactctggtttcaagcgtaaagccggcacgtccagcctgacggagtgcgtgttgaacaaggccacgaatgtcgcccactggacaacccccagtctcaaatgcattagagagccgaaatcttgtgacaaaactcacacatgcccaccgtgcccagcacctgaactcctggggggaccgtcagtcttcctcttccccccaaaacccaaggacaccctcatgatctcccggacccctgaggtcacatgcgtggtggtggacgtgagccacgaagaccctgaggtcaagttcaactggtacgtggacggcgtggaggtgcataatgccaagacaaagccgcgggaggagcagtacaacagcacgtaccgtgtggtcagcgtcctcaccgtcctgcaccaggactggctgaatggcaaggagtacaagtgcaaggtctccaacaaagccctcccagcccccatcgagaaaaccatctccaaagccaaagggcagccccgagaaccacaggtgtacaccctgcccccatcccgggatgagctgaccaagaaccaggtcagcctgacctgcctggtcaaaggcttctatcccagcgacatcgccgtggagtgggagagcaatgggcagccggagaacaactacaagaccacgcctcccgtgctggactccgacggctccttcttcctctacagcaagctcaccgtggacaagagcaggtggcagcaggggaacgtcttctcatgctccgtgatgcatgaggctctgcacaaccactacacgcagaagagcctctccctgtctcctggtaaataa

SEQ ID NO: 4 - protein, 557 aa, synthetic construct
  REGION 1..557: note = Description of Artificial Sequence: Synthetic polypeptide
MKWVTFISLLFLFSSAYSNIQMTQSPSSVSASVGDRVTITCRASQDISRWLAWYQQKPGKAPKLLIYAASSLQSGVPSRFSGSGSGTDFALTISSLQPEDFATYYCQQADSRFSITFGQGTRLEIKRGGGGSGGGGSGGGGSEVQLVQSGGGLVQPGGSLRLSCAASGFTFSSYSMNWVRQAPGKGLEWVSYISSSSSTIQYADSVKGRFTISRDNAKNSLYLQMNSLRDEDTAVYYCARGDYYYGMDVWGQGTTVTVSSITCPPPMSVEHADIWVKSYSLYSRERYICNSGFKRKAGTSSLTECVLNKATNVAHWTTPSLKCIREPKSCDKTHTCPPCPAPELLGGPSVFLFPPKPKDTLMISRTPEVTCVVVDVSHEDPEVKFNWYVDGVEVHNAKTKPREEQYNSTYRVVSVLTVLHQDWLNGKEYKCKVSNKALPAPIEKTISKAKGQPREPQVYTLPPSRDELTKNQVSLTCLVKGFYPSDIAVEWESNGQPENNYKTTPPVLDSDGSFFLYSKLTVDKSRWQQGNVFSCSVMHEALHNHYTQKSLSLSPGK

SEQ ID NO: 5 - DNA, 1134 bp, synthetic construct
  misc_feature 1..1134: note = Description of Artificial Sequence: Synthetic polynucleotide
  source 1..1134: mol_type = other DNA
atgaagtgggtgaccttcatcagcctgctgttcctgttctccagcgcctactcccagtccgctctgacccagcctgcttccgtgtccggctcccctggacagtccatcaccatctcctgtaccggcacctcctccgatgtgggcggctacaactacgtgtcctggtaccagcagcaccccggcaaagcccccaagctgatgatctatgacgtgtccaaccggccctccggcgtgtccaacaggttctccggctccaagtccggcaacaccgcctccctgacaatctccggcctgcaggccgaggatgaggctgactactactgctcctcctacacctcctcctccaccagggtgttcggcaccggcaccaaggtgaccgtgctgggaggtggcggatccggaggtggaggttctggtggaggtgggagtgaggtgcagctgctggagtccggaggcggactggtgcagcctggaggatccctgaggctgtcctgcgctgcctccggcttcaccttctcctcctacatcatgatgtgggtgaggcaggctcctggcaagggcctggagtgggtgtcctccatctacccctccggcggcatcaccttctacgccgataccgtgaagggcaggttcaccatctcccgggacaactccaagaacaccctgtacctgcagatgaactccctgagggctgaggacaccgccgtgtactactgcgccaggatcaagctgggcaccgtgaccacagtggactactggggacagggcaccctggtgaccgtgtcctccaactgggttaacgtaataagtgatttgaaaaaaattgaagatcttattcaatctatgcatattgatgctactttatatacggaaagtgatgttcaccccagttgcaaagtaacagcaatgaagtgctttctcttggagttacaagttatttcacttgagtccggagatgcaagtattcatgatacagtagaaaatctgatcatcctagcaaacgacagtttgtcttctaatgggaatgtaacagaatctggatgcaaagaatgtgaggaactggaggaaaaaaatattaaagaatttttgcagagttttgtacatattgtccaaatgttcatcaacacttcttaa

SEQ ID NO: 6 - protein, 377 aa, synthetic construct
  REGION 1..377: note = Description of Artificial Sequence: Synthetic polypeptide
MKWVTFISLLFLFSSAYSQSALTQPASVSGSPGQSITISCTGTSSDVGGYNYVSWYQQHPGKAPKLMIYDVSNRPSGVSNRFSGSKSGNTASLTISGLQAEDEADYYCSSYTSSSTRVFGTGTKVTVLGGGGSGGGGSGGGGSEVQLLESGGGLVQPGGSLRLSCAASGFTFSSYIMMWVRQAPGKGLEWVSSIYPSGGITFYADTVKGRFTISRDNSKNTLYLQMNSLRAEDTAVYYCARIKLGTVTTVDYWGQGTLVTVSSNWVNVISDLKKIEDLIQSMHIDATLYTESDVHPSCKVTAMKCFLLELQVISLESGDASIHDTVENLIILANDSLSSNGNVTESGCKECEELEEKNIKEFLQSFVHIVQMFINTS

SEQ ID NO: 7 - DNA, 1683 bp, synthetic construct
  misc_feature 1..1683: note = Description of Artificial Sequence: Synthetic polynucleotide
  source 1..1683: mol_type = other DNA
atgaagtgggtgaccttcatcagcctgctgttcctgttctccagcgcctactcccagtccgctctgacccagcctgcttccgtgtccggctcccctggacagtccatcaccatctcctgtaccggcacctcctccgatgtgggcggctacaactacgtgtcctggtaccagcagcaccccggcaaagcccccaagctgatgatctatgacgtgtccaaccggccctccggcgtgtccaacaggttctccggctccaagtccggcaacaccgcctccctgacaatctccggcctgcaggccgaggatgaggctgactactactgctcctcctacacctcctcctccaccagggtgttcggcaccggcaccaaggtgaccgtgctgggaggtggcggatccggaggtggaggttctggtggaggtgggagtgaggtgcagctgctggagtccggaggcggactggtgcagcctggaggatccctgaggctgtcctgcgctgcctccggcttcaccttctcctcctacatcatgatgtgggtgaggcaggctcctggcaagggcctggagtgggtgtcctccatctacccctccggcggcatcaccttctacgccgataccgtgaagggcaggttcaccatctcccgggacaactccaagaacaccctgtacctgcagatgaactccctgagggctgaggacaccgccgtgtactactgcgccaggatcaagctgggcaccgtgaccacagtggactactggggacagggcaccctggtgaccgtgtcctccatcacgtgccctccccccatgtccgtggaacacgcagacatctgggtcaagagctacagcttgtactccagggagcggtacatttgtaactctggtttcaagcgtaaagccggcacgtccagcctgacggagtgcgtgttgaacaaggccacgaatgtcgcccactggacaacccccagtctcaaatgcattagagagccgaaatcttgtgacaaaactcacacatgcccaccgtgcccagcacctgaactcctggggggaccgtcagtcttcctcttccccccaaaacccaaggacaccctcatgatctcccggacccctgaggtcacatgcgtggtggtggacgtgagccacgaagaccctgaggtcaagttcaactggtacgtggacggcgtggaggtgcataatgccaagacaaagccgcgggaggagcagtacaacagcacgtaccgtgtggtcagcgtcctcaccgtcctgcaccaggactggctgaatggcaaggagtacaagtgcaaggtctccaacaaagccctcccagcccccatcgagaaaaccatctccaaagccaaagggcagccccgagaaccacaggtgtacaccctgcccccatcccgggatgagctgaccaagaaccaggtcagcctgacctgcctggtcaaaggcttctatcccagcgacatcgccgtggagtgggagagcaatgggcagccggagaacaactacaagaccacgcctcccgtgctggactccgacggctccttcttcctctacagcaagctcaccgtggacaagagcaggtggcagcaggggaacgtcttctcatgctccgtgatgcatgaggctctgcacaaccactacacgcagaagagcctctccctgtctcctggtaaataa

SEQ ID NO: 8 - protein, 560 aa, synthetic construct
  REGION 1..560: note = Description of Artificial Sequence: Synthetic polypeptide
MKWVTFISLLFLFSSAYSQSALTQPASVSGSPGQSITISCTGTSSDVGGYNYVSWYQQHPGKAPKLMIYDVSNRPSGVSNRFSGSKSGNTASLTISGLQAEDEADYYCSSYTSSSTRVFGTGTKVTVLGGGGSGGGGSGGGGSEVQLLESGGGLVQPGGSLRLSCAASGFTFSSYIMMWVRQAPGKGLEWVSSIYPSGGITFYADTVKGRFTISRDNSKNTLYLQMNSLRAEDTAVYYCARIKLGTVTTVDYWGQGTLVTVSSITCPPPMSVEHADIWVKSYSLYSRERYICNSGFKRKAGTSSLTECVLNKATNVAHWTTPSLKCIREPKSCDKTHTCPPCPAPELLGGPSVFLFPPKPKDTLMISRTPEVTCVVVDVSHEDPEVKFNWYVDGVEVHNAKTKPREEQYNSTYRVVSVLTVLHQDWLNGKEYKCKVSNKALPAPIEKTISKAKGQPREPQVYTLPPSRDELTKNQVSLTCLVKGFYPSDIAVEWESNGQPENNYKTTPPVLDSDGSFFLYSKLTVDKSRWQQGNVFSCSVMHEALHNHYTQKSLSLSPGK

SEQ ID NO: 9 - DNA, 1131 bp, synthetic construct
  misc_feature 1..1131: note = Description of Artificial Sequence: Synthetic polynucleotide
  source 1..1131: mol_type = other DNA
atgacatggactctactattccttgccttccttcatcacttaacagggtcatgtgcccagtttgtgcttactcagccaaactctgtgtctacgaatctcggaagcacagtcaagctgtcttgcaaccgcagcactggtaacattggaaacaattatgtgaactggtaccagcagcatgaaggaagatctcccaccactctgatttattgggatgataggagaccagatggagttcctgacaggttctctggctccattgacagatcttccaactcagccctcctgacaatcaataatgtgcagactgaggatgaaactgactacttctgtcagtcttacagtagtggtatgtatattttcggcggtggaaccaagctcactgtcctaggaggtggcggatccggaggtggaggttctggtggaggtgggagtgaggttcagctgcagcagtctggggctgagctggtgaagcctggggcttcagtaaagttgtcctgcaaaacttctggttacaccttcagcaattactatatgagttggttgaagcagatgcctggacagaatattgagtggatcggaaacatttatggtggaaatggtggtgctggctataatcagaagttcaagggcaaggccacactgacagtggacaaatcttccagcacagcgtacatggatctcagcagcctgacatctgaggcctctgcagtctatttttgtgcaagggtcggacttcccggcctttttgattactggggccagggagtcatggtcacagtctcctcaaactgggtgaatgtaataagtgatttgaaaaaaattgaagatcttattcaatctatgcatattgatgctactttatatacggaaagtgatgttcaccccagttgcaaagtaacagcaatgaagtgctttctcttggagttacaagttatttcacttgagtccggagatgcaagtattcatgatacagtagaaaatctgatcatcctagcaaacgacagtttgtcttctaatgggaatgtaacagaatctggatgcaaagaatgtgaggaactggaggaaaaaaatattaaagaatttttgcagagttttgtacatattgtccaaatgttcatcaacacttcttaa

SEQ ID NO: 10 - protein, 376 aa, synthetic construct
  REGION 1..376: note = Description of Artificial Sequence: Synthetic polypeptide
MTWTLLFLAFLHHLTGSCAQFVLTQPNSVSTNLGSTVKLSCNRSTGNIGNNYVNWYQQHEGRSPTTLIYWDDRRPDGVPDRFSGSIDRSSNSALLTINNVQTEDETDYFCQSYSSGMYIFGGGTKLTVLGGGGSGGGGSGGGGSEVQLQQSGAELVKPGASVKLSCKTSGYTFSNYYMSWLKQMPGQNIEWIGNIYGGNGGAGYNQKFKGKATLTVDKSSSTAYMDLSSLTSEASAVYFCARVGLPGLFDYWGQGVMVTVSSNWVNVISDLKKIEDLIQSMHIDATLYTESDVHPSCKVTAMKCFLLELQVISLESGDASIHDTVENLIILANDSLSSNGNVTESGCKECEELEEKNIKEFLQSFVHIVQMFINTS

SEQ ID NO: 11 - DNA, 1683 bp, synthetic construct
  misc_feature 1..1683: note = Description of Artificial Sequence: Synthetic polynucleotide
  source 1..1683: mol_type = other DNA
atgacatggactctactattccttgccttccttcatcacttaacagggtcatgtgcccagtttgtgcttactcagccaaactctgtgtctacgaatctcggaagcacagtcaagctgtcttgcaaccgcagcactggtaacattggaaacaattatgtgaactggtaccagcagcatgaaggaagatctcccaccactctgatttattgggatgataggagaccagatggagttcctgacaggttctctggctccattgacagatcttccaactcagccctcctgacaatcaataatgtgcagactgaggatgaaactgactacttctgtcagtcttacagtagtggtatgtatattttcggcggtggaaccaagctcactgtcctaggaggtggcggatccggaggtggaggttctggtggaggtgggagtgaggttcagctgcagcagtctggggctgagctggtgaagcctggggcttcagtaaagttgtcctgcaaaacttctggttacaccttcagcaattactatatgagttggttgaagcagatgcctggacagaatattgagtggatcggaaacatttatggtggaaatggtggtgctggctataatcagaagttcaagggcaaggccacactgacagtggacaaatcttccagcacagcgtacatggatctcagcagcctgacatctgaggcctctgcagtctatttttgtgcaagggtcggacttcccggcctttttgattactggggccagggagtcatggtcacagtctcctcaatcacgtgccctccccccatgtccgtggaacacgcagacatctgggtcaagagctacagcttgtactccagggagcggtacatttgtaactctggtttcaagcgtaaagccggcacgtccagcctgacggagtgcgtgttgaacaaggccacgaatgtcgcccactggacaacccccagtctcaaatgcattagagaaccaagagggcccacaatcaagccctgtcctccatgcaaatgcccagcacctaacctcttgggtggaccatccgtcttcatcttccctccaaagatcaaggatgtactcatgatctccctgagccccatagtcacatgtgtggtggtggatgtgagcgaggatgacccagatgtccagatcagctggtttgtgaacaacgtggaagtacacacagctcagacacaaacccatagagaggattacaacagtactctccgggtggtcagtgccctccccatccagcaccaggactggatgagtggcaaggagttcaaatgcaaggtcaacaacaaagacctcccagcgcccatcgagagaaccatctcaaaacccaaagggtcagtaagagctccacaggtatatgtcttgcctccaccagaagaagagatgactaagaaacaggtcactctgacctgcatggtcacagacttcatgcctgaagacatttacgtggagtggaccaacaacgggaaaacagagctaaactacaagaacactgaaccagtcctggactctgatggttcttacttcatgtacagcaagctgagagtggaaaagaagaactgggtggaaagaaatagctactcctgttcagtggtccacgagggtctgcacaatcaccacacgactaagagcttctcccggactccaggtaaataa

SEQ ID NO: 12 - protein, 560 aa, synthetic construct
  REGION 1..560: note = Description of Artificial Sequence: Synthetic polypeptide
MTWTLLFLAFLHHLTGSCAQFVLTQPNSVSTNLGSTVKLSCNRSTGNIGNNYVNWYQQHEGRSPTTLIYWDDRRPDGVPDRFSGSIDRSSNSALLTINNVQTEDETDYFCQSYSSGMYIFGGGTKLTVLGGGGSGGGGSGGGGSEVQLQQSGAELVKPGASVKLSCKTSGYTFSNYYMSWLKQMPGQNIEWIGNIYGGNGGAGYNQKFKGKATLTVDKSSSTAYMDLSSLTSEASAVYFCARVGLPGLFDYWGQGVMVTVSSITCPPPMSVEHADIWVKSYSLYSRERYICNSGFKRKAGTSSLTECVLNKATNVAHWTTPSLKCIREPRGPTIKPCPPCKCPAPNLLGGPSVFIFPPKIKDVLMISLSPIVTCVVVDVSEDDPDVQISWFVNNVEVHTAQTQTHREDYNSTLRVVSALPIQHQDWMSGKEFKCKVNNKDLPAPIERTISKPKGSVRAPQVYVLPPPEEEMTKKQVTLTCMVTDFMPEDIYVEWTNNGKTELNYKNTEPVLDSDGSYFMYSKLRVEKKNWVERNSYSCSVVHEGLHNHHTTKSFSRTPGK

SEQ ID NO: 13 - DNA, 1692 bp, synthetic construct
  misc_feature 1..1692: note = Description of Artificial Sequence: Synthetic polynucleotide
  source 1..1692: mol_type = other DNA
atgaagtgggtgacctttatctccctgctgttcctgttttcctccgcctacagcatcgtgatgacccagtcccctagctccctgagcgctagcgtgggagaccgggtgaccatcacctgtcgggcctcccagagcatttccagctacctgaactggtaccagcagaagcccggcaaggcccctaagctgctgatttacgctgccagcagcctgcagtccggagtgcctcccaggtttagcggctccggatccggcaccgagttcaccctgaccatctcctccctgcagcccgaggacttcgccacctactactgtcagcaggccaacagctttccccccacctttggccaaggaaccaaggtggacatcaagaggaccgtggccggaggcggaggctccggcggcggcggctccggcggcggcggctccctggtgcagtccggcgctgaagtgaagaagcctggcgcctccgtgaaggtgtcctgcgaggcctccggctacaccttcaccaactactacatccactggctgaggcaggctcctggacagggcctggagtggatgggcatcatcaacccctccggaggctccaccacctacgcccagaagttccagggcaggatcaccatgacaagggacacctccaccaacaccctgtacatggaactgtcctccctccggtccgaggacaccgccatctactactgcgccaggagggattgcaggggccctagctgctacttcgcttactggggccagggaaccaccgtgaccgtgtcctccgcctccaccaagggcatcacgtgccctccccccatgtccgtggaacacgcagacatctgggtcaagagctacagcttgtactccagggagcggtacatttgtaactctggtttcaagcgtaaagccggcacgtccagcctgacggagtgcgtgttgaacaaggccacgaatgtcgcccactggacaacccccagtctcaaatgcattagagagccgaaatcttgtgacaaaactcacacatgcccaccgtgcccagcacctgaactcctggggggaccgtcagtcttcctcttccccccaaaacccaaggacaccctcatgatctcccggacccctgaggtcacatgcgtggtggtggacgtgagccacgaagaccctgaggtcaagttcaactggtacgtggacggcgtggaggtgcataatgccaagacaaagccgcgggaggagcagtacaacagcacgtaccgtgtggtcagcgtcctcaccgtcctgcaccaggactggctgaatggcaaggagtacaagtgcaaggtctccaacaaagccctcccagcccccatcgagaaaaccatctccaaagccaaagggcagccccgagaaccacaggtgtacaccctgcccccatcccgggatgagctgaccaagaaccaggtcagcctgacctgcctggtcaaaggcttctatcccagcgacatcgccgtggagtgggagagcaatgggcagccggagaacaactacaagaccacgcctcccgtgctggactccgacggctccttcttcctctacagcaagctcaccgtggacaagagcaggtggcagcaggggaacgtcttctcatgctccgtgatgcatgaggctctgcacaaccactacacgcagaagagcctctccctgtctcctggtaaataa

SEQ ID NO: 14 - protein, 563 aa, synthetic construct
  REGION 1..563: note = Description of Artificial Sequence: Synthetic polypeptide
MKWVTFISLLFLFSSAYSIVMTQSPSSLSASVGDRVTITCRASQSISSYLNWYQQKPGKAPKLLIYAASSLQSGVPPRFSGSGSGTEFTLTISSLQPEDFATYYCQQANSFPPTFGQGTKVDIKRTVAGGGGSGGGGSGGGGSLVQSGAEVKKPGASVKVSCEASGYTFTNYYIHWLRQAPGQGLEWMGIINPSGGSTTYAQKFQGRITMTRDTSTNTLYMELSSLRSEDTAIYYCARRDCRGPSCYFAYWGQGTTVTVSSASTKGITCPPPMSVEHADIWVKSYSLYSRERYICNSGFKRKAGTSSLTECVLNKATNVAHWTTPSLKCIREPKSCDKTHTCPPCPAPELLGGPSVFLFPPKPKDTLMISRTPEVTCVVVDVSHEDPEVKFNWYVDGVEVHNAKTKPREEQYNSTYRVVSVLTVLHQDWLNGKEYKCKVSNKALPAPIEKTISKAKGQPREPQVYTLPPSRDELTKNQVSLTCLVKGFYPSDIAVEWESNGQPENNYKTTPPVLDSDGSFFLYSKLTVDKSRWQQGNVFSCSVMHEALHNHYTQKSLSLSPGK

SEQ ID NO: 15 - DNA, 1689 bp, synthetic construct
  misc_feature 1..1689: note = Description of Artificial Sequence: Synthetic polynucleotide
  source 1..1689: mol_type = other DNA
atgaagtgggtaacctttatttcccttctttttctctttagctcggcttattccgacatcatgatgacccagtccccttcctccctgtccgtgagcgctggcgagaaggctaccatcagctgcaagtcctcccagtccctgttcaacagcaacgccaagaccaactacctgaactggtacctgcagaagcccggccagtcccccaagctgctgatctattacgctagcaccaggcataccggcgtgcccgacaggtttaggggatccggcagcggcaccgacttcaccctgaccatctccagcgtgcaggacgaggacctcgctttctactactgccagcaatggtacgattacccttacaccttcggcgctggcaccaaggtggagattaagaggggcggaggcggatccggcggcggcggctccggcggcggaggctcccagattcagctgcaggagtccggccctggactggtcaaccctagccagtccctgagcctgtcctgttccgtgacaggctatagcatcaccagcggctacggctggaactggatcaggcagtttcccggccagaaagtggagtggatgggcttcatctactacgagggctccacctactataacccctccatcaagtcccggatcagcatcaccagggatacctccaagaaccagttcttcctgcaagtcaactccgtgaccaccgaagacaccgccacctactactgcgccaggcagacaggctacttcgactactggggccagggcacaatggtgaccgtcagcagcgccatcacgtgccctccccccatgtccgtggaacacgcagacatctgggtcaagagctacagcttgtactccagggagcggtacatttgtaactctggtttcaagcgtaaagccggcacgtccagcctgacggagtgcgtgttgaacaaggccacgaatgtcgcccactggacaacccccagtctcaaatgcattagagaaccaagagggcccacaatcaagccctgtcctccatgcaaatgcccagcacctaacctcttgggtggaccatccgtcttcatcttccctccaaagatcaaggatgtactcatgatctccctgagccccatagtcacatgtgtggtggtggatgtgagcgaggatgacccagatgtccagatcagctggtttgtgaacaacgtggaagtacacacagctcagacacaaacccatagagaggattacaacagtactctccgggtggtcagtgccctccccatccagcaccaggactggatgagtggcaaggagttcaaatgcaaggtcaacaacaaagacctcccagcgcccatcgagagaaccatctcaaaacccaaagggtcagtaagagctccacaggtatatgtcttgcctccaccagaagaagagatgactaagaaacaggtcactctgacctgcatggtcacagacttcatgcctgaagacatttacgtggagtggaccaacaacgggaaaacagagctaaactacaagaacactgaaccagtcctggactctgatggttcttacttcatgtacagcaagctgagagtggaaaagaagaactgggtggaaagaaatagctactcctgttcagtggtccacgagggtctgcacaatcaccacacgactaagagcttctcccggactccaggtaaataa

SEQ ID NO: 16 - protein, 562 aa, synthetic construct
  REGION 1..562: note = Description of Artificial Sequence: Synthetic polypeptide
MKWVTFISLLFLFSSAYSDIMMTQSPSSLSVSAGEKATISCKSSQSLFNSNAKTNYLNWYLQKPGQSPKLLIYYASTRHTGVPDRFRGSGSGTDFTLTISSVQDEDLAFYYCQQWYDYPYTFGAGTKVEIKRGGGGSGGGGSGGGGSQIQLQESGPGLVNPSQSLSLSCSVTGYSITSGYGWNWIRQFPGQKVEWMGFIYYEGSTYYNPSIKSRISITRDTSKNQFFLQVNSVTTEDTATYYCARQTGYFDYWGQGTMVTVSSAITCPPPMSVEHADIWVKSYSLYSRERYICNSGFKRKAGTSSLTECVLNKATNVAHWTTPSLKCIREPRGPTIKPCPPCKCPAPNLLGGPSVFIFPPKIKDVLMISLSPIVTCVVVDVSEDDPDVQISWFVNNVEVHTAQTQTHREDYNSTLRVVSALPIQHQDWMSGKEFKCKVNNKDLPAPIERTISKPKGSVRAPQVYVLPPPEEEMTKKQVTLTCMVTDFMPEDIYVEWTNNGKTELNYKNTEPVLDSDGSYFMYSKLRVEKKNWVERNSYSCSVVHEGLHNHHTTKSFSRTPGK

SEQ ID NO: 17 - DNA, 1131 bp, synthetic construct
  misc_feature 1..1131: note = Description of Artificial Sequence: Synthetic polynucleotide
  source 1..1131: mol_type = other DNA
atggaatggagctgggtgttcctgttctttctgtccgtgaccaccggtgtccactccctgcctgtgctgactcaaccaccctcggtgtctgaagtccccgggcagagggtcaccatttcctgttctggaggcatctccaacatcggaagcaatgctgtaaactggtaccagcacttcccaggaaaggctcccaaactcctcatctattataatgatctgctgccctcaggggtctctgaccgattctctgcctccaagtctggcacctcagcctccctggccatcagtgggctccggtccgaggatgaggctgattattactgtgcagcatgggatgacaatctgagtgcttatgtcttcgcaactgggaccaaggtcaccgtcctgagtggaggtggcggatccggaggtggaggttctggtggaggtgggagtcaggttcagctggtgcagtctggggctgaggtgaagaagcctggggcctcagtgaaggtctcctgcaaggcttctggttacacctttaccagctatggtatcagctgggtgcgacaggcccctggacaagggcttgagtggatgggatggatcagcgcttacaatggtaacacaaactatgcacagaagctccagggcagagtcaccatgaccacagacacatccacgagcacagcctacatggagctgaggagcctgagatctgacgacacggccgtgtattactgtgcgagagggttatacggtgacgaggactactggggccagggaaccctggtcaccgtgagctcaaactgggttaacgtaataagtgatttgaaaaaaattgaagatcttattcaatctatgcatattgatgctactttatatacggaaagtgatgttcaccccagttgcaaagtaacagcaatgaagtgctttctcttggagttacaagttatttcacttgagtccggagatgcaagtattcatgatacagtagaaaatctgatcatcctagcaaacgacagtttgtcttctaatgggaatgtaacagaatctggatgcaaagaatgtgaggaactggaggaaaaaaatattaaagaatttttgcagagttttgtacatattgtccaaatgttcatcaacacttcttaa

SEQ ID NO: 18 - protein, 376 aa, synthetic construct
  REGION 1..376: note = Description of Artificial Sequence: Synthetic polypeptide
MEWSWVFLFFLSVTTGVHSLPVLTQPPSVSEVPGQRVTISCSGGISNIGSNAVNWYQHFPGKAPKLLIYYNDLLPSGVSDRFSASKSGTSASLAISGLRSEDEADYYCAAWDDNLSAYVFATGTKVTVLSGGGGSGGGGSGGGGSQVQLVQSGAEVKKPGASVKVSCKASGYTFTSYGISWVRQAPGQGLEWMGWISAYNGNTNYAQKLQGRVTMTTDTSTSTAYMELRSLRSDDTAVYYCARGLYGDEDYWGQGTLVTVSSNWVNVISDLKKIEDLIQSMHIDATLYTESDVHPSCKVTAMKCFLLELQVISLESGDASIHDTVENLIILANDSLSSNGNVTESGCKECEELEEKNIKEFLQSFVHIVQMFINTS

SEQ ID NO: 19 - DNA, 768 bp, synthetic construct
  misc_feature 1..768: note = Description of Artificial Sequence: Synthetic polynucleotide
  source 1..768: mol_type = other DNA
atgaagtgggtgaccttcatcagcctgctgttcctgttctccagcgcctactcccaggtgcagctggtggagtccggaggaggcctggtggagcctggaggatccctgaggctgtcctgtgccgccagcggcatcatcttcaagatcaacgacatgggctggtatcggcaggcccctggcaaaaggagggagtgggtggccgcttccacaggaggcgatgaggccatctacagggactccgtgaaggacaggttcaccatctccagggacgccaagaactccgtgttcctgcagatgaactccctgaagcccgaggataccgccgtgtactactgcaccgccgtgatctccaccgatagggacggcaccgagtggaggaggtactggggccagggcacacaggtgactgtgtcctccggcggcaactgggttaacgtaataagtgatttgaaaaaaattgaagatcttattcaatctatgcatattgatgctactttatatacggaaagtgatgttcaccccagttgcaaagtaacagcaatgaagtgctttctcttggagttacaagttatttcacttgagtccggagatgcaagtattcatgatacagtagaaaatctgatcatcctagcaaacgacagtttgtcttctaatgggaatgtaacagaatctggatgcaaagaatgtgaggaactggaggaaaaaaatattaaagaatttttgcagagttttgtacatattgtccaaatgttcatcaacacttcttaa

SEQ ID NO: 20 - protein, 255 aa, synthetic construct
  REGION 1..255: note = Description of Artificial Sequence: Synthetic polypeptide
MKWVTFISLLFLFSSAYSQVQLVESGGGLVEPGGSLRLSCAASGIIFKINDMGWYRQAPGKRREWVAASTGGDEAIYRDSVKDRFTISRDAKNSVFLQMNSLKPEDTAVYYCTAVISTDRDGTEWRRYWGQGTQVTVSSGGNWVNVISDLKKIEDLIQSMHIDATLYTESDVHPSCKVTAMKCFLLELQVISLESGDASIHDTVENLIILANDSLSSNGNVTESGCKECEELEEKNIKEFLQSFVHIVQMFINTS

SEQ ID NO: 21 - DNA, 1317 bp, synthetic construct
  misc_feature 1..1317: note = Description of Artificial Sequence: Synthetic polynucleotide
  source 1..1317: mol_type = other DNA
atgaagtgggtgaccttcatcagcctgctgttcctgttctccagcgcctactcccaggtgcagctggtggagtccggaggaggcctggtggagcctggaggatccctgaggctgtcctgtgccgccagcggcatcatcttcaagatcaacgacatgggctggtatcggcaggcccctggcaaaaggagggagtgggtggccgcttccacaggaggcgatgaggccatctacagggactccgtgaaggacaggttcaccatctccagggacgccaagaactccgtgttcctgcagatgaactccctgaagcccgaggataccgccgtgtactactgcaccgccgtgatctccaccgatagggacggcaccgagtggaggaggtactggggccagggcacacaggtgactgtgtcctccggcggcatcacgtgtcctcctcctatgtccgtggaacacgcagacatctgggtcaagagctacagcttgtactccagggagcggtacatttgtaactctggtttcaagcgtaaagccggcacgtccagcctgacggagtgcgtgttgaacaaggccacgaatgtcgcccactggacaacccccagtctcaaatgcattagagaaccaagagggcccacaatcaagccctgtcctccatgcaaatgcccagcacctaacctcttgggtggaccatccgtcttcatcttccctccaaagatcaaggatgtactcatgatctccctgagccccatagtcacatgtgtggtggtggatgtgagcgaggatgacccagatgtccagatcagctggtttgtgaacaacgtggaagtacacacagctcagacacaaacccatagagaggattacaacagtactctccgggtggtcagtgccctccccatccagcaccaggactggatgagtggcaaggagttcaaatgcaaggtcaacaacaaagacctcccagcgcccatcgagagaaccatctcaaaacccaaagggtcagtaagagctccacaggtatatgtcttgcctccaccagaagaagagatgactaagaaacaggtcactctgacctgcatggtcacagacttcatgcctgaagacatttacgtggagtggaccaacaacgggaaaacagagctaaactacaagaacactgaaccagtcctggactctgatggttcttacttcatgtacagcaagctgagagtggaaaagaagaactgggtggaaagaaatagctactcctgttcagtggtccacgagggtctgcacaatcaccacacgactaagagcttctcccggactccaggtaaa

SEQ ID NO: 22 - protein, 439 aa, synthetic construct
  REGION 1..439: note = Description of Artificial Sequence: Synthetic polypeptide
MKWVTFISLLFLFSSAYSQVQLVESGGGLVEPGGSLRLSCAASGIIFKINDMGWYRQAPGKRREWVAASTGGDEAIYRDSVKDRFTISRDAKNSVFLQMNSLKPEDTAVYYCTAVISTDRDGTEWRRYWGQGTQVTVSSGGITCPPPMSVEHADIWVKSYSLYSRERYICNSGFKRKAGTSSLTECVLNKATNVAHWTTPSLKCIREPRGPTIKPCPPCKCPAPNLLGGPSVFIFPPKIKDVLMISLSPIVTCVVVDVSEDDPDVQISWFVNNVEVHTAQTQTHREDYNSTLRVVSALPIQHQDWMSGKEFKCKVNNKDLPAPIERTISKPKGSVRAPQVYVLPPPEEEMTKKQVTLTCMVTDFMPEDIYVEWTNNGKTELNYKNTEPVLDSDGSYFMYSKLRVEKKNWVERNSYSCSVVHEGLHNHHTTKSFSRTPGK

SEQ ID NO: 23 - DNA, 1119 bp, synthetic construct
  misc_feature 1..1119: note = Description of Artificial Sequence: Synthetic polynucleotide
  source 1..1119: mol_type = other DNA
atgaagtgggtgaccttcatcagcctgctgttcctgttctccagcgcctactccaacatccagatgacccagtccccttccgccatgagcgcttccgtgggcgacagggtgaccatcacctgcaaggcctcccaggacatccacaggtacctgtcctggttccagcagaagcccggcaaggtgcccaagcacctgatctacagggctaacaggctggtgtccggcgtgccttccaggttttccggctccggctccggcaccgagttcaccctgaccatctccagcctgcagcccgaggacttcgccacctactactgcctgcagtacgacgagttcccctacaccttcggcggcggcaccaaggtggagatcaagggaggtggcggatccggaggtggaggttctggtggaggtgggagtcagatgcagctggtacagtccggcgccgaggtgaagaagaccggctccagcgtgaaggtgtcctgcaaggcctccggcttcaacatcaaggactactacctgcactgggtgaggcaggcccctggacaagccctggagtggatgggctggatcgaccccgacaacggcgacaccgagtacgcccagaagttccaggacagggtgaccatcaccagggacaggtccatgagcaccgcctacatggagctgtcctccctgaggtccgaggacaccgccatgtactactgcaacgccgcctacggctcctcctcctaccccatggactactggggccagggcaccaccgtgaccgtgaactgggttaacgtaataagtgatttgaaaaaaattgaagatcttattcaatctatgcatattgatgctactttatatacggaaagtgatgttcaccccagttgcaaagtaacagcaatgaagtgctttctcttggagttacaagttatttcacttgagtccggagatgcaagtattcatgatacagtagaaaatctgatcatcctagcaaacgacagtttgtcttctaatgggaatgtaacagaatctggatgcaaagaatgtgaggaactggaggaaaaaaatattaaagaatttttgcagagttttgtacatattgtccaaatgttcatcaacacttcttaa

SEQ ID NO: 24 - protein, 372 aa, synthetic construct
  REGION 1..372: note = Description of Artificial Sequence: Synthetic polypeptide
MKWVTFISLLFLFSSAYSNIQMTQSPSAMSASVGDRVTITCKASQDIHRYLSWFQQKPGKVPKHLIYRANRLVSGVPSRFSGSGSGTEFTLTISSLQPEDFATYYCLQYDEFPYTFGGGTKVEIKGGGGSGGGGSGGGGSQMQLVQSGAEVKKTGSSVKVSCKASGFNIKDYYLHWVRQAPGQALEWMGWIDPDNGDTEYAQKFQDRVTITRDRSMSTAYMELSSLRSEDTAMYYCNAAYGSSSYPMDYWGQGTTVTVNWVNVISDLKKIEDLIQSMHIDATLYTESDVHPSCKVTAMKCFLLELQVISLESGDASIHDTVENLIILANDSLSSNGNVTESGCKECEELEEKNIKEFLQSFVHIVQMFINTS

SEQ ID NO: 25 - DNA, 1668 bp, synthetic construct
  misc_feature 1..1668: note = Description of Artificial Sequence: Synthetic polynucleotide
  source 1..1668: mol_type = other DNA
atgaagtgggtgaccttcatcagcctgctgttcctgttctccagcgcctactccaacatccagatgacccagtccccttccgccatgagcgcttccgtgggcgacagggtgaccatcacctgcaaggcctcccaggacatccacaggtacctgtcctggttccagcagaagcccggcaaggtgcccaagcacctgatctacagggctaacaggctggtgtccggcgtgccttccaggttttccggctccggctccggcaccgagttcaccctgaccatctccagcctgcagcccgaggacttcgccacctactactgcctgcagtacgacgagttcccctacaccttcggcggcggcaccaaggtggagatcaagggaggtggcggatccggaggtggaggttctggtggaggtgggagtcagatgcagctggtacagtccggcgccgaggtgaagaagaccggctccagcgtgaaggtgtcctgcaaggcctccggcttcaacatcaaggactactacctgcactgggtgaggcaggcccctggacaagccctggagtggatgggctggatcgaccccgacaacggcgacaccgagtacgcccagaagttccaggacagggtgaccatcaccagggacaggtccatgagcaccgcctacatggagctgtcctccctgaggtccgaggacaccgccatgtactactgcaacgccgcctacggctcctcctcctaccccatggactactggggccagggcaccaccgtgaccgtgatcacgtgtcctcctcctatgtccgtggaacacgcagacatctgggtcaagagctacagcttgtactccagggagcggtacatttgtaactctggtttcaagcgtaaagccggcacgtccagcctgacggagtgcgtgttgaacaaggccacgaatgtcgcccactggacaacccccagtctcaaatgcattagagagccgaaatcttgtgacaaaactcacacatgcccaccgtgcccagcacctgaactcctggggggaccgtcagtcttcctcttccccccaaaacccaaggacaccctcatgatctcccggacccctgaggtcacatgcgtggtggtggacgtgagccacgaagaccctgaggtcaagttcaactggtacgtggacggcgtggaggtgcataatgccaagacaaagccgcgggaggagcagtacaacagcacgtaccgtgtggtcagcgtcctcaccgtcctgcaccaggactggctgaatggcaaggagtacaagtgcaaggtctccaacaaagccctcccagcccccatcgagaaaaccatctccaaagccaaagggcagccccgagaaccacaggtgtacaccctgcccccatcccgggatgagctgaccaagaaccaggtcagcctgacctgcctggtcaaaggcttctatcccagcgacatcgccgtggagtgggagagcaatgggcagccggagaacaactacaagaccacgcctcccgtgctggactccgacggctccttcttcctctacagcaagctcaccgtggacaagagcaggtggcagcaggggaacgtcttctcatgctccgtgatgcatgaggctctgcacaaccactacacgcagaagagcctctccctgtctcctggtaaataa

SEQ ID NO: 26 - protein, 555 aa, synthetic construct
  REGION 1..555: note = Description of Artificial Sequence: Synthetic polypeptide
MKWVTFISLLFLFSSAYSNIQMTQSPSAMSASVGDRVTITCKASQDIHRYLSWFQQKPGKVPKHLIYRANRLVSGVPSRFSGSGSGTEFTLTISSLQPEDFATYYCLQYDEFPYTFGGGTKVEIKGGGGSGGGGSGGGGSQMQLVQSGAEVKKTGSSVKVSCKASGFNIKDYYLHWVRQAPGQALEWMGWIDPDNGDTEYAQKFQDRVTITRDRSMSTAYMELSSLRSEDTAMYYCNAAYGSSSYPMDYWGQGTTVTVITCPPPMSVEHADIWVKSYSLYSRERYICNSGFKRKAGTSSLTECVLNKATNVAHWTTPSLKCIREPKSCDKTHTCPPCPAPELLGGPSVFLFPPKPKDTLMISRTPEVTCVVVDVSHEDPEVKFNWYVDGVEVHNAKTKPREEQYNSTYRVVSVLTVLHQDWLNGKEYKCKVSNKALPAPIEKTISKAKGQPREPQVYTLPPSRDELTKNQVSLTCLVKGFYPSDIAVEWESNGQPENNYKTTPPVLDSDGSFFLYSKLTVDKSRWQQGNVFSCSVMHEALHNHYTQKSLSLSPGK

SEQ ID NO: 27 - DNA, 744 bp, synthetic construct
  misc_feature 1..744: note = Description of Artificial Sequence: Synthetic polynucleotide
  source 1..744: mol_type = other DNA
atgaagtgggtgaccttcatcagcctgctgttcctgttctccagcgcctactccaccgccaaggagccctgcatggccaagttcggccctctgccctccaagtggcagatggcctcctccgagcctccctgtgtgaacaaggtgtccgactggaagctggagatcctgcagaacggcctgtacctgatctacggccaggtggcccccaacgccaactacaacgacgtggcccccttcgaggtgcggctgtacaagaacaaggacatgatccagaccctgaccaacaagtccaagatccagaacgtgggcggcacctatgagctgcacgtgggcgacaccatcgacctgatcttcaactccgagcaccaggtgctgaagaacaacacctactggggcatcaactgggttaacgtaataagtgatttgaaaaaaattgaagatcttattcaatctatgcatattgatgctactttatatacggaaagtgatgttcaccccagttgcaaagtaacagcaatgaagtgctttctcttggagttacaagttatttcacttgagtccggagatgcaagtattcatgatacagtagaaaatctgatcatcctagcaaacgacagtttgtcttctaatgggaatgtaacagaatctggatgcaaagaatgtgaggaactggaggaaaaaaatattaaagaatttttgcagagttttgtacatattgtccaaatgttcatcaacacttcttaa

SEQ ID NO: 28 - protein, 247 aa, synthetic construct
  REGION 1..247: note = Description of Artificial Sequence: Synthetic polypeptide
MKWVTFISLLFLFSSAYSTAKEPCMAKFGPLPSKWQMASSEPPCVNKVSDWKLEILQNGLYLIYGQVAPNANYNDVAPFEVRLYKNKDMIQTLTNKSKIQNVGGTYELHVGDTIDLIFNSEHQVLKNNTYWGINWVNVISDLKKIEDLIQSMHIDATLYTESDVHPSCKVTAMKCFLLELQVISLESGDASIHDTVENLIILANDSLSSNGNVTESGCKECEELEEKNIKEFLQSFVHIVQMFINTS

SEQ ID NO: 29 - DNA, 1293 bp, synthetic construct
  misc_feature 1..1293: note = Description of Artificial Sequence: Synthetic polynucleotide
  source 1..1293: mol_type = other DNA
atgaagtgggtgaccttcatcagcctgctgttcctgttctccagcgcctactccaccgccaaggagccctgcatggccaagttcggccctctgccctccaagtggcagatggcctcctccgagcctccctgtgtgaacaaggtgtccgactggaagctggagatcctgcagaacggcctgtacctgatctacggccaggtggcccccaacgccaactacaacgacgtggcccccttcgaggtgcggctgtacaagaacaaggacatgatccagaccctgaccaacaagtccaagatccagaacgtgggcggcacctatgagctgcacgtgggcgacaccatcgacctgatcttcaactccgagcaccaggtgctgaagaacaacacctactggggcatcatcacgtgtcctcctcctatgtccgtggaacacgcagacatctgggtcaagagctacagcttgtactccagggagcggtacatttgtaactctggtttcaagcgtaaagccggcacgtccagcctgacggagtgcgtgttgaacaaggccacgaatgtcgcccactggacaacccccagtctcaaatgcattagagagccgaaatcttgtgacaaaactcacacatgcccaccgtgcccagcacctgaactcctggggggaccgtcagtcttcctcttccccccaaaacccaaggacaccctcatgatctcccggacccctgaggtcacatgcgtggtggtggacgtgagccacgaagaccctgaggtcaagttcaactggtacgtggacggcgtggaggtgcataatgccaagacaaagccgcgggaggagcagtacaacagcacgtaccgtgtggtcagcgtcctcaccgtcctgcaccaggactggctgaatggcaaggagtacaagtgcaaggtctccaacaaagccctcccagcccccatcgagaaaaccatctccaaagccaaagggcagccccgagaaccacaggtgtacaccctgcccccatcccgggatgagctgaccaagaaccaggtcagcctgacctgcctggtcaaaggcttctatcccagcgacatcgccgtggagtgggagagcaatgggcagccggagaacaactacaagaccacgcctcccgtgctggactccgacggctccttcttcctctacagcaagctcaccgtggacaagagcaggtggcagcaggggaacgtcttctcatgctccgtgatgcatgaggctctgcacaaccactacacgcagaagagcctctccctgtctcctggtaaataa

SEQ ID NO: 30 - protein, 430 aa, synthetic construct
  REGION 1..430: note = Description of Artificial Sequence: Synthetic polypeptide
MKWVTFISLLFLFSSAYSTAKEPCMAKFGPLPSKWQMASSEPPCVNKVSDWKLEILQNGLYLIYGQVAPNANYNDVAPFEVRLYKNKDMIQTLTNKSKIQNVGGTYELHVGDTIDLIFNSEHQVLKNNTYWGIITCPPPMSVEHADIWVKSYSLYSRERYICNSGFKRKAGTSSLTECVLNKATNVAHWTTPSLKCIREPKSCDKTHTCPPCPAPELLGGPSVFLFPPKPKDTLMISRTPEVTCVVVDVSHEDPEVKFNWYVDGVEVHNAKTKPREEQYNSTYRVVSVLTVLHQDWLNGKEYKCKVSNKALPAPIEKTISKAKGQPREPQVYTLPPSRDELTKNQVSLTCLVKGFYPSDIAVEWESNGQPENNYKTTPPVLDSDGSFFLYSKLTVDKSRWQQGNVFSCSVMHEALHNHYTQKSLSLSPGK

SEQ ID NO: 31 - DNA, 1131 bp, synthetic construct
  misc_feature 1..1131: note = Description of Artificial Sequence: Synthetic polynucleotide
  source 1..1131: mol_type = other DNA
atgaagtgggtgaccttcatcagcctgctgttcctgttctccagcgcctactccgagatcgtgctgacccagtcccctgctaccctgtccctgtcccctggcgagagggctaccctgtcctgcagggccaggcaatccatctccaactacctgcactggtaccagcagaaacctggccaggcccccaggctgctgatctactacgcctcccagtccatctccggcatccctgacaggttcagcggatccggctccggcaccgacttcaccctgaccatctccaggctggagcctgaggacttcgccgtgtactactgccagcagtccaactcctggcctctgaccttcggccagggcaccaaggtggagatcaagcggggaggtggcggatccggaggtggaggttctggtggaggtgggagtgaggtgcagctggtgcagtccggcgccgaagtgaagaagcccggagcctccgtgaaggtgtcctgcaaggcctccggctacaccttcaccaggtactggatgcactgggtgaggcaggcccctggacagggactggagtggatcggcgccatctaccccggcaactccgacacctcctacaaccagaagttcaagggcaaggccaccatcaccgccgacacctccaccaacaccgcctacatggagctgtcctccctgaggtccgaggacaccgccgtgtactactgcgctaggggcgaggagatcggcgtgaggaggtggttcgcctactggggacagggcaccctggtgaccgtgtccagcaactgggttaacgtaataagtgatttgaaaaaaattgaagatcttattcaatctatgcatattgatgctactttatatacggaaagtgatgttcaccccagttgcaaagtaacagcaatgaagtgctttctcttggagttacaagttatttcacttgagtccggagatgcaagtattcatgatacagtagaaaatctgatcatcctagcaaacgacagtttgtcttctaatgggaatgtaacagaatctggatgcaaagaatgtgaggaactggaggaaaaaaatattaaagaatttttgcagagttttgtacatattgtccaaatgttcatcaacacttcttaa

SEQ ID NO: 32 - protein, 376 aa, synthetic construct
  REGION 1..376: note = Description of Artificial Sequence: Synthetic polypeptide
MKWVTFISLLFLFSSAYSEIVLTQSPATLSLSPGERATLSCRARQSISNYLHWYQQKPGQAPRLLIYYASQSISGIPDRFSGSGSGTDFTLTISRLEPEDFAVYYCQQSNSWPLTFGQGTKVEIKRGGGGSGGGGSGGGGSEVQLVQSGAEVKKPGASVKVSCKASGYTFTRYWMHWVRQAPGQGLEWIGAIYPGNSDTSYNQKFKGKATITADTSTNTAYMELSSLRSEDTAVYYCARGEEIGVRRWFAYWGQGTLVTVSSNWVNVISDLKKIEDLIQSMHIDATLYTESDVHPSCKVTAMKCFLLELQVISLESGDASIHDTVENLIILANDSLSSNGNVTESGCKECEELEEKNIKEFLQSFVHIVQMFINTS

SEQ ID NO: 33 - DNA, 1680 bp, synthetic construct
  misc_feature 1..1680: note = Description of Artificial Sequence: Synthetic polynucleotide
  source 1..1680: mol_type = other DNA
atgaagtgggtgaccttcatcagcctgctgttcctgttctccagcgcctactccgagatcgtgctgacccagtcccctgctaccctgtccctgtcccctggcgagagggctaccctgtcctgcagggccaggcaatccatctccaactacctgcactggtaccagcagaaacctggccaggcccccaggctgctgatctactacgcctcccagtccatctccggcatccctgacaggttcagcggatccggctccggcaccgacttcaccctgaccatctccaggctggagcctgaggacttcgccgtgtactactgccagcagtccaactcctggcctctgaccttcggccagggcaccaaggtggagatcaagcggggaggtggcggatccggaggtggaggttctggtggaggtgggagtgaggtgcagctggtgcagtccggcgccgaagtgaagaagcccggagcctccgtgaaggtgtcctgcaaggcctccggctacaccttcaccaggtactggatgcactgggtgaggcaggcccctggacagggactggagtggatcggcgccatctaccccggcaactccgacacctcctacaaccagaagttcaagggcaaggccaccatcaccgccgacacctccaccaacaccgcctacatggagctgtcctccctgaggtccgaggacaccgccgtgtactactgcgctaggggcgaggagatcggcgtgaggaggtggttcgcctactggggacagggcaccctggtgaccgtgtccagcatcacgtgtcctcctcctatgtccgtggaacacgcagacatctgggtcaagagctacagcttgtactccagggagcggtacatttgtaactctggtttcaagcgtaaagccggcacgtccagcctgacggagtgcgtgttgaacaaggccacgaatgtcgcccactggacaacccccagtctcaaatgcattagagagccgaaatcttgtgacaaaactcacacatgcccaccgtgcccagcacctgaactcctggggggaccgtcagtcttcctcttccccccaaaacccaaggacaccctcatgatctcccggacccctgaggtcacatgcgtggtggtggacgtgagccacgaagaccctgaggtcaagttcaactggtacgtggacggcgtggaggtgcataatgccaagacaaagccgcgggaggagcagtacaacagcacgtaccgtgtggtcagcgtcctcaccgtcctgcaccaggactggctgaatggcaaggagtacaagtgcaaggtctccaacaaagccctcccagcccccatcgagaaaaccatctccaaagccaaagggcagccccgagaaccacaggtgtacaccctgcccccatcccgggatgagctgaccaagaaccaggtcagcctgacctgcctggtcaaaggcttctatcccagcgacatcgccgtggagtgggagagcaatgggcagccggagaacaactacaagaccacgcctcccgtgctggactccgacggctccttcttcctctacagcaagctcaccgtggacaagagcaggtggcagcaggggaacgtcttctcatgctccgtgatgcatgaggctctgcacaaccactacacgcagaagagcctctccctgtctcctggtaaataa

SEQ ID NO: 34 - protein, 559 aa, synthetic construct
  REGION 1..559: note = Description of Artificial Sequence: Synthetic polypeptide
MKWVTFISLLFLFSSAYSEIVLTQSPATLSLSPGERATLSCRARQSISNYLHWYQQKPGQAPRLLIYYASQSISGIPDRFSGSGSGTDFTLTISRLEPEDFAVYYCQQSNSWPLTFGQGTKVEIKRGGGGSGGGGSGGGGSEVQLVQSGAEVKKPGASVKVSCKASGYTFTRYWMHWVRQAPGQGLEWIGAIYPGNSDTSYNQKFKGKATITADTSTNTAYMELSSLRSEDTAVYYCARGEEIGVRRWFAYWGQGTLVTVSSITCPPPMSVEHADIWVKSYSLYSRERYICNSGFKRKAGTSSLTECVLNKATNVAHWTTPSLKCIREPKSCDKTHTCPPCPAPELLGGPSVFLFPPKPKDTLMISRTPEVTCVVVDVSHEDPEVKFNWYVDGVEVHNAKTKPREEQYNSTYRVVSVLTVLHQDWLNGKEYKCKVSNKALPAPIEKTISKAKGQPREPQVYTLPPSRDELTKNQVSLTCLVKGFYPSDIAVEWESNGQPENNYKTTPPVLDSDGSFFLYSKLTVDKSRWQQGNVFSCSVMHEALHNHYTQKSLSLSPGK

SEQ ID NO: 35 - DNA, 1662 bp, synthetic construct
  misc_feature 1..1662: note = Description of Artificial Sequence: Synthetic polynucleotide
  source 1..1662: mol_type = other DNA
atgaagtgggtgaccttcatcagcctgctgttcctgttctccagcgcctactccgacatccagatgacccagtcccctgcttccctgtccgcttccgtgggcgacagggtgaccatcacctgcctggcctcccagaccatcgacacctggctggcctggtacctgcagaagcccggcaagtccccccagctgctgatctacgccgctaccaacctggccgacggcgtgcctagcaggttttccggctccggctccggcaccgacttctccttcaccatctcctccctgcagcccgaggacttcgccacctactactgccagcaggtgtactcctcccccttcaccttcggccagggcaccaagctggagatcaagggaggtggcggatccggaggtggaggttctggtggaggtgggagtcagatccagctggtgcagtccggcggcgaagtgaaaaagcccggcgccagcgtgagggtgtcctgtaaggcctccggctactccttcaccgactacaacgtgtactgggtgaggcagtcccccggcaagggactggagtggatcggctacatcgacccctacaacggcatcaccatctacgaccagaacttcaagggcaaggccaccctgaccgtggacaagtccacctccacagcctacatggagctgtcctccctgaggtccgaggacaccgccgtgtacttctgcgccagggacgtgaccaccgctctggacttctggggacagggcaccaccgtgaccgtgagctccatcacgtgtcctcctcctatgtccgtggaacacgcagacatctgggtcaagagctacagcttgtactccagggagcggtacatttgtaactctggtttcaagcgtaaagccggcacgtccagcctgacggagtgcgtgttgaacaaggccacgaatgtcgcccactggacaacccccagtctcaaatgcattagagagccgaaatcttgtgacaaaactcacacatgcccaccgtgcccagcacctgaactcctggggggaccgtcagtcttcctcttccccccaaaacccaaggacaccctcatgatctcccggacccctgaggtcacatgcgtggtggtggacgtgagccacgaagaccctgaggtcaagttcaactggtacgtggacggcgtggaggtgcataatgccaagacaaagccgcgggaggagcagtacaacagcacgtaccgtgtggtcagcgtcctcaccgtcctgcaccaggactggctgaatggcaaggagtacaagtgcaaggtctccaacaaagccctcccagcccccatcgagaaaaccatctccaaagccaaagggcagccccgagaaccacaggtgtacaccctgcccccatcccgggatgagctgaccaagaaccaggtcagcctgacctgcctggtcaaaggcttctatcccagcgacatcgccgtggagtgggagagcaatgggcagccggagaacaactacaagaccacgcctcccgtgctggactccgacggctccttcttcctctacagcaagctcaccgtggacaagagcaggtggcagcaggggaacgtcttctcatgctccgtgatgcatgaggctctgcacaaccactacacgcagaagagcctctccctgtctcctggtaaa

SEQ ID NO: 36 - protein, 554 aa, synthetic construct
  REGION 1..554: note = Description of Artificial Sequence: Synthetic polypeptide
MKWVTFISLLFLFSSAYSDIQMTQSPASLSASVGDRVTITCLASQTIDTWLAWYLQKPGKSPQLLIYAATNLADGVPSRFSGSGSGTDFSFTISSLQPEDFATYYCQQVYSSPFTFGQGTKLEIKGGGGSGGGGSGGGGSQIQLVQSGGEVKKPGASVRVSCKASGYSFTDYNVYWVRQSPGKGLEWIGYIDPYNGITIYDQNFKGKATLTVDKSTSTAYMELSSLRSEDTAVYFCARDVTTALDFWGQGTTVTVSSITCPPPMSVEHADIWVKSYSLYSRERYICNSGFKRKAGTSSLTECVLNKATNVAHWTTPSLKCIREPKSCDKTHTCPPCPAPELLGGPSVFLFPPKPKDTLMISRTPEVTCVVVDVSHEDPEVKFNWYVDGVEVHNAKTKPREEQYNSTYRVVSVLTVLHQDWLNGKEYKCKVSNKALPAPIEKTISKAKGQPREPQVYTLPPSRDELTKNQVSLTCLVKGFYPSDIAVEWESNGQPENNYKTTPPVLDSDGSFFLYSKLTVDKSRWQQGNVFSCSVMHEALHNHYTQKSLSLSPGK

SEQ ID NO: 37 - DNA, 1137 bp, synthetic construct
  misc_feature 1..1137: note = Description of Artificial Sequence: Synthetic polynucleotide
  source 1..1137: mol_type = other DNA
atggattttcaggtgcagattatcagcttcctgctaatcagtgcttcagtcataatgtcaagaggacaggtgcagctggttcagagcggtgcggaagttaaaaagccgggctcttccgtgaaagttagctgcaaagcgtctggttataccttcaccgactacaacatgcactgggtccgccaggccccaggccagggtctggaatggatcggttatatttacccgtacaacggtggcacgggatataaccagaaattcaaatccaaagctaccatcactgcggacgaaagcaccaacaccgcatatatggaattgtcttctctgcgtagcgaagataccgcggtttactattgcgctcgtggtcgtccagcgatggattactggggtcagggcaccctggtgaccgtgagctctggcggaggcggatctggtggtggcggatccggtggaggcggaagcgatatccagatgacccagtccccgagctccctgtctgccagcgtgggcgaccgcgtgactatcacctgccgtgcgtccgaaagcgtggataactacggcatttcctttatgaactggttccagcagaaaccgggtaaagccccgaaactgctgatttatgcggcctctaaccagggcagcggtgtgccgagccgcttttccggcagcggttcggggaccgatttcactctgaccatttctagcctgcagccagatgacttcgcgacctactactgccaacagtctaaagaagttccgtggaccttcggtcagggtaccaaagttgaaattaaaaactgggttaacgtaataagtgatttgaaaaaaattgaagatcttattcaatctatgcatattgatgctactttatatacggaaagtgatgttcaccccagttgcaaagtaacagcaatgaagtgctttctcttggagttacaagttatttcacttgagtccggagatgcaagtattcatgatacagtagaaaatctgatcatcctagcaaacgacagtttgtcttctaatgggaatgtaacagaatctggatgcaaagaatgtgaggaactggaggaaaaaaatattaaagaatttttgcagagttttgtacatattgtccaaatgttcatcaacacttcttaa

SEQ ID NO: 38 - protein, 378 aa, synthetic construct
  REGION 1..378: note = Description of Artificial Sequence: Synthetic polypeptide
MDFQVQIISFLLISASVIMSRGQVQLVQSGAEVKKPGSSVKVSCKASGYTFTDYNMHWVRQAPGQGLEWIGYIYPYNGGTGYNQKFKSKATITADESTNTAYMELSSLRSEDTAVYYCARGRPAMDYWGQGTLVTVSSGGGGSGGGGSGGGGSDIQMTQSPSSLSASVGDRVTITCRASESVDNYGISFMNWFQQKPGKAPKLLIYAASNQGSGVPSRFSGSGSGTDFTLTISSLQPDDFATYYCQQSKEVPWTFGQGTKVEIKNWVNVISDLKKIEDLIQSMHIDATLYTESDVHPSCKVTAMKCFLLELQVISLESGDASIHDTVENLIILANDSLSSNGNVTESGCKECEELEEKNIKEFLQSFVHIVQMFINTS

SEQ ID NO: 39 - DNA, 1686 bp, synthetic construct
  misc_feature 1..1686: note = Description of Artificial Sequence: Synthetic polynucleotide
  source 1..1686: mol_type = other DNA
atggattttcaggtgcagattatcagcttcctgctaatcagtgcttcagtcataatgtcaagaggacaggtgcagctggttcagagcggtgcggaagttaaaaagccgggctcttccgtgaaagttagctgcaaagcgtctggttataccttcaccgactacaacatgcactgggtccgccaggccccaggccagggtctggaatggatcggttatatttacccgtacaacggtggcacgggatataaccagaaattcaaatccaaagctaccatcactgcggacgaaagcaccaacaccgcatatatggaattgtcttctctgcgtagcgaagataccgcggtttactattgcgctcgtggtcgtccagcgatggattactggggtcagggcaccctggtgaccgtgagctctggcggaggcggatctggtggtggcggatccggtggaggcggaagcgatatccagatgacccagtccccgagctccctgtctgccagcgtgggcgaccgcgtgactatcacctgccgtgcgtccgaaagcgtggataactacggcatttcctttatgaactggttccagcagaaaccgggtaaagccccgaaactgctgatttatgcggcctctaaccagggcagcggtgtgccgagccgcttttccggcagcggttcggggaccgatttcactctgaccatttctagcctgcagccagatgacttcgcgacctactactgccaacagtctaaagaagttccgtggaccttcggtcagggtaccaaagttgaaattaaaatcacgtgtcctcctcctatgtccgtggaacacgcagacatctgggtcaagagctacagcttgtactccagggagcggtacatttgtaactctggtttcaagcgtaaagccggcacgtccagcctgacggagtgcgtgttgaacaaggccacgaatgtcgcccactggacaacccccagtctcaaatgcattagagagccgaaatcttgtgacaaaactcacacatgcccaccgtgcccagcacctgaactcctggggggaccgtcagtcttcctcttccccccaaaacccaaggacaccctcatgatctcccggacccctgaggtcacatgcgtggtggtggacgtgagccacgaagaccctgaggtcaagttcaactggtacgtggacggcgtggaggtgcataatgccaagacaaagccgcgggaggagcagtacaacagcacgtaccgtgtggtcagcgtcctcaccgtcctgcaccaggactggctgaatggcaaggagtacaagtgcaaggtctccaacaaagccctcccagcccccatcgagaaaaccatctccaaagccaaagggcagccccgagaaccacaggtgtacaccctgcccccatcccgggatgagctgaccaagaaccaggtcagcctgacctgcctggtcaaaggcttctatcccagcgacatcgccgtggagtgggagagcaatgggcagccggagaacaactacaagaccacgcctcccgtgctggactccgacggctccttcttcctctacagcaagctcaccgtggacaagagcaggtggcagcaggggaacgtcttctcatgctccgtgatgcatgaggctctgcacaaccactacacgcagaagagcctctccctgtctcctggtaaataa

SEQ ID NO: 40 - protein, 561 aa, synthetic construct
  REGION 1..561: note = Description of Artificial Sequence: Synthetic polypeptide
MDFQVQIISFLLISASVIMSRGQVQLVQSGAEVKKPGSSVKVSCKASGYTFTDYNMHWVRQAPGQGLEWIGYIYPYNGGTGYNQKFKSKATITADESTNTAYMELSSLRSEDTAVYYCARGRPAMDYWGQGTLVTVSSGGGGSGGGGSGGGGSDIQMTQSPSSLSASVGDRVTITCRASESVDNYGISFMNWFQQKPGKAPKLLIYAASNQGSGVPSRFSGSGSGTDFTLTISSLQPDDFATYYCQQSKEVPWTFGQGTKVEIKITCPPPMSVEHADIWVKSYSLYSRERYICNSGFKRKAGTSSLTECVLNKATNVAHWTTPSLKCIREPKSCDKTHTCPPCPAPELLGGPSVFLFPPKPKDTLMISRTPEVTCVVVDVSHEDPEVKFNWYVDGVEVHNAKTKPREEQYNSTYRVVSVLTVLHQDWLNGKEYKCKVSNKALPAPIEKTISKAKGQPREPQVYTLPPSRDELTKNQVSLTCLVKGFYPSDIAVEWESNGQPENNYKTTPPVLDSDGSFFLYSKLTVDKSRWQQGNVFSCSVMHEALHNHYTQKSLSLSPGK

SEQ ID NO: 41 - DNA, 1626 bp, synthetic construct
  misc_feature 1..1626: note = Description of Artificial Sequence: Synthetic polynucleotide
  source 1..1626: mol_type = other DNA
atgaagtgggtgaccttcatcagcctgctgttcctgttctccagcgcctactccatgaagtgggtgaccttcatcagcctgctgttcctgttctccagcgcctactccgatttagtgtttctgttcgacggctccatgtctttacagcccgatgagttccagaagattttagacttcatgaaggacgtgatgaagaaactgtccaacaccagctaccagttcgctgccgtgcagttctccacctcctacaagaccgagttcgacttctccgactacgtgaagcggaaggaccccgatgctttactgaagcacgtcaagcacatgctgctgctcaccaacacctttggcgccatcaactacgtggccaccgaggtgtttcgtgaggaactgggagctcggcccgatgccaccaaggtgctgattatcatcaccgacggcgaagccaccgatagcggaaacatcgatgccgccaaggacatcatccggtacattatcggcatcggcaagcacttccagaccaaggagagccaagagactttacacaagttcgcctccaagcccgcttccgagttcgtgtgcattttagacaccttcgagtgtttaaaggatttatttaccgagctgcagaagaagatctacgtgattgagggcaccagcaagcaagatctgacctccttcaacatggagctgtccagcagcggcatttccgctgatttatctcgtggccacgccatcacgtgtcctcctcctatgtccgtggaacacgcagacatctgggtcaagagctacagcttgtactccagggagcggtacatttgtaactctggtttcaagcgtaaagccggcacgtccagcctgacggagtgcgtgttgaacaaggccacgaatgtcgcccactggacaacccccagtctcaaatgcattagagagccgaaatcttgtgacaaaactcacacatgcccaccgtgcccagcacctgaactcctggggggaccgtcagtcttcctcttccccccaaaacccaaggacaccctcatgatctcccggacccctgaggtcacatgcgtggtggtggacgtgagccacgaagaccctgaggtcaagttcaactggtacgtggacggcgtggaggtgcataatgccaagacaaagccgcgggaggagcagtacaacagcacgtaccgtgtggtcagcgtcctcaccgtcctgcaccaggactggctgaatggcaaggagtacaagtgcaaggtctccaacaaagccctcccagcccccatcgagaaaaccatctccaaagccaaagggcagccccgagaaccacaggtgtacaccctgcccccatcccgggatgagctgaccaagaaccaggtcagcctgacctgcctggtcaaaggcttctatcccagcgacatcgccgtggagtgggagagcaatgggcagccggagaacaactacaagaccacgcctcccgtgctggactccgacggctccttcttcctctacagcaagctcaccgtggacaagagcaggtggcagcaggggaacgtcttctcatgctccgtgatgcatgaggctctgcacaaccactacacgcagaagagcctctccctgtctcctggtaaataa

SEQ ID NO: 42 - protein, 523 aa, synthetic construct
  REGION 1..523: note = Description of Artificial Sequence: Synthetic polypeptide
MKWVTFISLLFLFSSAYSDLVFLFDGSMSLQPDEFQKILDFMKDVMKKLSNTSYQFAAVQFSTSYKTEFDFSDYVKRKDPDALLKHVKHMLLLTNTFGAINYVATEVFREELGARPDATKVLIIITDGEATDSGNIDAAKDIIRYIIGIGKHFQTKESQETLHKFASKPASEFVCILDTFECLKDLFTELQKKIYVIEGTSKQDLTSFNMELSSSGISADLSRGHAITCPPPMSVEHADIWVKSYSLYSRERYICNSGFKRKAGTSSLTECVLNKATNVAHWTTPSLKCIREPKSCDKTHTCPPCPAPELLGGPSVFLFPPKPKDTLMISRTPEVTCVVVDVSHEDPEVKFNWYVDGVEVHNAKTKPREEQYNSTYRVVSVLTVLHQDWLNGKEYKCKVSNKALPAPIEKTISKAKGQPREPQVYTLPPSRDELTKNQVSLTCLVKGFYPSDIAVEWESNGQPENNYKTTPPVLDSDGSFFLYSKLTVDKSRWQQGNVFSCSVMHEALHNHYTQKSLSLSPGK

SEQ ID NO: 43 - DNA, 2457 bp, synthetic construct
  misc_feature 1..2457: note = Description of Artificial Sequence: Synthetic polynucleotide
  source 1..2457: mol_type = other DNA
atgaagtgggtgaccttcatcagcctgctgttcctgttctccagcgcctactccagcggcgtgttccagctgcagctgcaagagtttatcaacgagaggggcgtgctggcttccggtcgtccttgtgagcccggttgtaggacctttttccgggtgtgtttaaagcattttcaagctgtggtgtcccccggaccttgtaccttcggcaccgtgtccacccccgttctgggcaccaactccttcgccgttcgtgacgacagctccggaggaggtcgtaatcctttacagctgcctttcaactttacttggcccggcaccttctccctcatcatcgaagcttggcatgcccccggtgacgatctgcggcccgaagctctgccccccgatgctttaatcagcaagattgccattcaaggttctttagccgtgggccagaactggctgctggacgagcagaccagcacactcactcgtctgaggtactcctatcgtgtgatctgcagcgacaactactacggcgacaattgcagccggctgtgcaagaagaggaacgaccacttcggccattacgtctgccagcccgacggcaatttatcttgtctgcccggttggaccggcgagtactgtcagcagcccatctgtttaagcggctgccacgagcagaacggctactgcagcaagcccgctgagtgtctgtgtaggcccggctggcaaggtaggctgtgcaacgagtgcatcccccacaatggctgtcggcacggcacttgttccaccccttggcagtgcacttgtgacgagggctggggaggtttattctgcgaccaagatctgaactactgcacccaccacagcccttgtaagaacggagctacttgttccaacagcggccagaggtcctacacttgtacttgtaggcccggttacaccggcgtcgactgcgaactggaactgagcgaatgcgatagcaacccttgtcgtaacggcggcagctgcaaggaccaagaagacggctaccactgtttatgccctcccggatactacggtttacactgcgagcactccacactgtcttgtgccgactccccttgtttcaacggcggaagctgtcgtgagaggaaccaaggtgccaactacgcttgtgagtgccctcccaacttcaccggctccaactgcgagaagaaggtggatcgttgcacctccaacccttgcgccaacggcggccagtgtttaaataggggcccttcccggatgtgtcgttgtcgtcccggttttaccggcacctactgcgagctgcacgtcagcgattgcgcccggaatccttgcgctcacggcggaacttgtcacgatttagagaacggtttaatgtgcacttgtcccgctggattcagcggtcgtaggtgtgaggtgaggacctccatcgacgcttgtgccagcagcccttgcttcaatcgtgccacttgttacaccgatttatccaccgacaccttcgtgtgcaactgcccctacggcttcgtgggatctcgttgcgagttccccgttggcctgcctcctagctttccctggatcacgtgtcctcctcctatgtccgtggaacacgcagacatctgggtcaagagctacagcttgtactccagggagcggtacatttgtaactctggtttcaagcgtaaagccggcacgtccagcctgacggagtgcgtgttgaacaaggccacgaatgtcgcccactggacaacccccagtctcaaatgcattagagagccgaaatcttgtgacaaaactcacacatgcccaccgtgcccagcacctgaactcctggggggaccgtcagtcttcctcttccccccaaaacccaaggacaccctcatgatctcccggacccctgaggtcacatgcgtggtggtggacgtgagccacgaagaccctgaggtcaagttcaactggtacgtggacggcgtggaggtgcataatgccaagacaaagccgcgggaggagcagtacaacagcacgtaccgtgtggtcagcgtcctcaccgtcctgcaccaggactggctgaatggcaaggagtacaagtgcaaggtctccaacaaagccctcccagcccccatcgagaaaaccatctccaaagccaaagggcagccccgagaaccacaggtgtacaccctgcccccatcccgggatgagctgaccaagaaccaggtcagcctgacctgcctggtcaaaggcttctatcccagcgacatcgccgtggagtgggagagcaatgggcagccggagaacaactacaagaccacgcctcccgtgctggactccgacggctccttcttcctctacagcaagctcaccgtggacaagagcaggtggcagcaggggaacgtcttctcatgctccgtgatgcatgaggctctgcacaaccactacacgcagaagagcctctccctgtctcctggtaaataa

SEQ ID NO: 44 - protein, 818 aa, synthetic construct
  REGION 1..818: note = Description of Artificial Sequence: Synthetic polypeptide
MKWVTFISLLFLFSSAYSSGVFQLQLQEFINERGVLASGRPCEPGCRTFFRVCLKHFQAVVSPGPCTFGTVSTPVLGTNSFAVRDDSSGGGRNPLQLPFNFTWPGTFSLIIEAWHAPGDDLRPEALPPDALISKIAIQGSLAVGQNWLLDEQTSTLTRLRYSYRVICSDNYYGDNCSRLCKKRNDHFGHYVCQPDGNLSCLPGWTGEYCQQPICLSGCHEQNGYCSKPAECLCRPGWQGRLCNECIPHNGCRHGTCSTPWQCTCDEGWGGLFCDQDLNYCTHHSPCKNGATCSNSGQRSYTCTCRPGYTGVDCELELSECDSNPCRNGGSCKDQEDGYHCLCPPGYYGLHCEHSTLSCADSPCFNGGSCRERNQGANYACECPPNFTGSNCEKKVDRCTSNPCANGGQCLNRGPSRMCRCRPGFTGTYCELHVSDCARNPCAHGGTCHDLENGLMCTCPAGFSGRRCEVRTSIDACASSPCFNRATCYTDLSTDTFVCNCPYGFVGSRCEFPVGLPPSFPWITCPPPMSVEHADIWVKSYSLYSRERYICNSGFKRKAGTSSLTECVLNKATNVAHWTTPSLKCIREPKSCDKTHTCPPCPAPELLGGPSVFLFPPKPKDTLMISRTPEVTCVVVDVSHEDPEVKFNWYVDGVEVHNAKTKPREEQYNSTYRVVSVLTVLHQDWLNGKEYKCKVSNKALPAPIEKTISKAKGQPREPQVYTLPPSRDELTKNQVSLTCLVKGFYPSDIAVEWESNGQPENNYKTTPPVLDSDGSFFLYSKLTVDKSRWQQGNVFSCSVMHEALHNHYTQKSLSLSPGK

SEQ ID NO: 45 - DNA, 1701 bp, synthetic construct
  misc_feature 1..1701: note = Description of Artificial Sequence: Synthetic polynucleotide
  source 1..1701: mol_type = other DNA
atggaatggagctgggtctttctcttcttcctgtcagtaaccaccggtgtccactcctcctatgtgctgactcagcctccctccgcgtccgggtctcctggacagtcagtcaccatctcctgcactggaaccagcagtgacgttggtaataataactatgtctcctggtaccaacagcacccaggcaaagcccccaaactcatgatttatgatgtcagtaatcggccctcaggggtttctactcgcttctctggctccaagtctggcaacacggcctccctgaccatctctgggctccaggctgaggacgaggctgattattactgcagctcatatacaaccagcagtacttatgtcttcggaactgggaccaagctgaccgtcctggggcagccaaaggcgggaggtggcggatccggaggtggaggttctggtggaggtgggagtctggtgcaatctggggctgaggtgaagaagcctggggcctcagtgaaggtctcctgcaaggcttctggatacaccttcaccggctactatatgcactgggtgcgacaggcccctggacaagggcttgagtggatgggatggatcaaccctaacagtggtggcacaaactatgcacagaagttccagggcagagtcaccatgaccaggaacacctccataagcacagcctacatggagttgagcagcctgagatctgacgacacggccgtgtattactgtgcgagagagatgtattactatggttcggggtacaactggttcgacccctggggccagggaaccctggtcaccgtgagctcaatcacgtgtcctcctcctatgtccgtggaacacgcagacatctgggtcaagagctacagcttgtactccagggagcggtacatttgtaactctggtttcaagcgtaaagccggcacgtccagcctgacggagtgcgtgttgaacaaggccacgaatgtcgcccactggacaacccccagtctcaaatgcattagagagccgaaatcttgtgacaaaactcacacatgcccaccgtgcccagcacctgaactcctggggggaccgtcagtcttcctcttccccccaaaacccaaggacaccctcatgatctcccggacccctgaggtcacatgcgtggtggtggacgtgagccacgaagaccctgaggtcaagttcaactggtacgtggacggcgtggaggtgcataatgccaagacaaagccgcgggaggagcagtacaacagcacgtaccgtgtggtcagcgtcctcaccgtcctgcaccaggactggctgaatggcaaggagtacaagtgcaaggtctccaacaaagccctcccagcccccatcgagaaaaccatctccaaagccaaagggcagccccgagaaccacaggtgtacaccctgcccccatcccgggatgagctgaccaagaaccaggtcagcctgacctgcctggtcaaaggcttctatcccagcgacatcgccgtggagtgggagagcaatgggcagccggagaacaactacaagaccacgcctcccgtgctggactccgacggctccttcttcctctacagcaagctcaccgtggacaagagcaggtggcagcaggggaacgtcttctcatgctccgtgatgcatgaggctctgcacaaccactacacgcagaagagcctctccctgtctcctggtaaataa

SEQ ID NO: 46 - protein, 566 aa, synthetic construct
  REGION 1..566: note = Description of Artificial Sequence: Synthetic polypeptide
MEWSWVFLFFLSVTTGVHSSYVLTQPPSASGSPGQSVTISCTGTSSDVGNNNYVSWYQQHPGKAPKLMIYDVSNRPSGVSTRFSGSKSGNTASLTISGLQAEDEADYYCSSYTTSSTYVFGTGTKLTVLGQPKAGGGGSGGGGSGGGGSLVQSGAEVKKPGASVKVSCKASGYTFTGYYMHWVRQAPGQGLEWMGWINPNSGGTNYAQKFQGRVTMTRNTSISTAYMELSSLRSDDTAVYYCAREMYYYGSGYNWFDPWGQGTLVTVSSITCPPPMSVEHADIWVKSYSLYSRERYICNSGFKRKAGTSSLTECVLNKATNVAHWTTPSLKCIREPKSCDKTHTCPPCPAPELLGGPSVFLFPPKPKDTLMISRTPEVTCVVVDVSHEDPEVKFNWYVDGVEVHNAKTKPREEQYNSTYRVVSVLTVLHQDWLNGKEYKCKVSNKALPAPIEKTISKAKGQPREPQVYTLPPSRDELTKNQVSLTCLVKGFYPSDIAVEWESNGQPENNYKTTPPVLDSDGSFFLYSKLTVDKSRWQQGNVFSCSVMHEALHNHYTQKSLSLSPGK

SEQ ID NO: 47 - DNA, 1665 bp, synthetic construct
  misc_feature 1..1665: note = Description of Artificial Sequence: Synthetic polynucleotide
  source 1..1665: mol_type = other DNA
atgaagtgggtgaccttcatcagcctgctgttcctgttctccagcgcctactcctacatccacgtgacccagtccccctcctctttaagcgtgagcatcggagatcgtgtgaccatcaactgccagacctcccaaggtgtgggctccgatttacactggtaccagcacaagcccggtcgggcccccaagctgctgatccaccacaccagctccgtggaggatggcgtgccctctcgtttctccggctccggcttccatacctccttcaatttaaccatcagcgatttacaagctgacgacatcgccacctactactgccaagttctccagttcttcggccggggctctcgtctgcatatcaagggaggcggcggatccggcggcggaggcagcggcggaggcggatctcgtgctcatctggtgcagagcggaaccgccatgaagaagcccggtgctagcgtgcgggtgtcttgtcagaccagcggatacaccttcaccgcccacattttattctggtttcgtcaagctcccggtcgtggactggaatgggtgggctggatcaagccccagtatggcgccgtgaactttggcggcggctttcgtgatcgggtgactttaactcgtgacgtgtatcgggagatcgcctacatggacattaggggtttaaagcccgacgataccgccgtgtactactgcgctcgtgatcgttcctacggcgatagcagctgggctttagatgcttggggccaaggtaccacagtgtggtccgccatcacgtgtcctcctcctatgtccgtggaacacgcagacatctgggtcaagagctacagcttgtactccagggagcggtacatttgtaactctggtttcaagcgtaaagccggcacgtccagcctgacggagtgcgtgttgaacaaggccacgaatgtcgcccactggacaacccccagtctcaaatgcattagagagccgaaatcttgtgacaaaactcacacatgcccaccgtgcccagcacctgaactcctggggggaccgtcagtcttcctcttccccccaaaacccaaggacaccctcatgatctcccggacccctgaggtcacatgcgtggtggtggacgtgagccacgaagaccctgaggtcaagttcaactggtacgtggacggcgtggaggtgcataatgccaagacaaagccgcgggaggagcagtacaacagcacgtaccgtgtggtcagcgtcctcaccgtcctgcaccaggactggctgaatggcaaggagtacaagtgcaaggtctccaacaaagccctcccagcccccatcgagaaaaccatctccaaagccaaagggcagccccgagaaccacaggtgtacaccctgcccccatcccgggatgagctgaccaagaaccaggtcagcctgacctgcctggtcaaaggcttctatcccagcgacatcgccgtggagtgggagagcaatgggcagccggagaacaactacaagaccacgcctcccgtgctggactccgacggctccttcttcctctacagcaagctcaccgtggacaagagcaggtggcagcaggggaacgtcttctcatgctccgtgatgcatgaggctctgcacaaccactacacgcagaagagcctctccctgtctcctggtaaataa

SEQ ID NO: 48 - DNA, 1680 bp, synthetic construct
  misc_feature 1..1680: note = Description of Artificial Sequence: Synthetic polynucleotide
  source 1..1680: mol_type = other DNA
atgaagtgggtgaccttcatcagcctgctgttcctgttctccagcgcctactccgtggtgatgacccagtccccttccaccctgtccgcttccgtgggcgacaccatcaccatcacctgcagggcctcccagtccatcgagacctggctggcctggtaccagcagaagcccggcaaggcccccaagctgctgatctacaaggcctccaccctgaagaccggcgtgccctccaggttttccggatccggctccggcaccgagttcaccctgaccatcagcggcctgcagttcgacgacttcgccacctaccactgccagcactacgccggctactccgccacctttggacagggcaccagggtggagatcaagggaggtggcggatccggaggtggaggttctggtggaggtgggagtgaggtgcagctggtggaatccggaggcggcctggtgaaagctggcggaagcctgatcctgagctgcggcgtgtccaacttcaggatctccgcccacaccatgaactgggtgaggagggtgcctggaggaggactggagtgggtggccagcatctccacctcctccacctacagggactacgccgacgccgtgaagggcaggttcaccgtgagcagggacgacctggaggacttcgtgtacctgcagatgcacaagatgcgggtggaggacaccgccatctactactgcgccaggaagggctccgacaggctgtccgacaacgacccctttgacgcctggggccctggaaccgtggtgacagtgtcccccatcacgtgtcctcctcctatgtccgtggaacacgcagacatctgggtcaagagctacagcttgtactccagggagcggtacatttgtaactctggtttcaagcgtaaagccggcacgtccagcctgacggagtgcgtgttgaacaaggccacgaatgtcgcccactggacaacccccagtctcaaatgcattagagagccgaaatcttgtgacaaaactcacacatgcccaccgtgcccagcacctgaactcctggggggaccgtcagtcttcctcttccccccaaaacccaaggacaccctcatgatctcccggacccctgaggtcacatgcgtggtggtggacgtgagccacgaagaccctgaggtcaagttcaactggtacgtggacggcgtggaggtgcataatgccaagacaaagccgcgggaggagcagtacaacagcacgtaccgtgtggtcagcgtcctcaccgtcctgcaccaggactggctgaatggcaaggagtacaagtgcaaggtctccaacaaagccctcccagcccccatcgagaaaaccatctccaaagccaaagggcagccccgagaaccacaggtgtacaccctgcccccatcccgggatgagctgaccaagaaccaggtcagcctgacctgcctggtcaaaggcttctatcccagcgacatcgccgtggagtgggagagcaatgggcagccggagaacaactacaagaccacgcctcccgtgctggactccgacggctccttcttcctctacagcaagctcaccgtggacaagagcaggtggcagcaggggaacgtcttctcatgctccgtgatgcatgaggctctgcacaaccactacacgcagaagagcctctccctgtctcctggtaaataa

SEQ ID NO: 49 - DNA, 1674 bp, synthetic construct
  misc_feature 1..1674: note = Description of Artificial Sequence: Synthetic polynucleotide
  source 1..1674: mol_type = other DNA
atgaagtgggtgaccttcatcagcctgctgttcctgttctccagcgcctactcctcctccctgacccagagccccggaacactctccctctcccccggtgagaccgctatcatctcttgtaggaccagccagtacggctctttagcttggtatcaacagaggcccggccaagctcctaggctggtcatttacagcggcagcacaagggccgccggcatccccgataggttctccggctcccggtggggccccgattacaatttaacaatctccaatttagagtccggagacttcggcgtctactactgccagcagtacgagttcttcggccaaggtaccaaagtgcaagttgatatcaagggcggcggaggctccggcggcggcggatccggcggaggaggatcccaagttaggctgtcccagagcggaggccagatgaagaagcccggtgactccatgcggatcagctgtcgtgccagcggctacgagttcatcaactgccccatcaactggattcgtctggcccccggtaagcggcccgaatggatgggctggatgaaacctcgtcacggcgctgtgtcctacgctcgtcagctgcaaggtcgtgtgaccatgactcgtgacatgtacagcgagaccgcctttttagagctgaggtctttaacctccgacgacaccgctgtgtacttctgcacccggggcaagtactgcaccgctcgggactactacaactgggacttcgagcactggggccaaggtacacccgtgacagtgtcctccatcacgtgtcctcctcctatgtccgtggaacacgcagacatctgggtcaagagctacagcttgtactccagggagcggtacatttgtaactctggtttcaagcgtaaagccggcacgtccagcctgacggagtgcgtgttgaacaaggccacgaatgtcgcccactggacaacccccagtctcaaatgcattagagagccgaaatcttgtgacaaaactcacacatgcccaccgtgcccagcacctgaactcctggggggaccgtcagtcttcctcttccccccaaaacccaaggacaccctcatgatctcccggacccctgaggtcacatgcgtggtggtggacgtgagccacgaagaccctgaggtcaagttcaactggtacgtggacggcgtggaggtgcataatgccaagacaaagccgcgggaggagcagtacaacagcacgtaccgtgtggtcagcgtcctcaccgtcctgcaccaggactggctgaatggcaaggagtacaagtgcaaggtctccaacaaagccctcccagcccccatcgagaaaaccatctccaaagccaaagggcagccccgagaaccacaggtgtacaccctgcccccatcccgggatgagctgaccaagaaccaggtcagcctgacctgcctggtcaaaggcttctatcccagcgacatcgccgtggagtgggagagcaatgggcagccggagaacaactacaagaccacgcctcccgtgctggactccgacggctccttcttcctctacagcaagctcaccgtggacaagagcaggtggcagcaggggaacgtcttctcatgctccgtgatgcatgaggctctgcacaaccactacacgcagaagagcctctccctgtctcctggtaaataa

SEQ ID NO: 50 - DNA, 1716 bp, synthetic construct
  misc_feature 1..1716: note = Description of Artificial Sequence: Synthetic polynucleotide
  source 1..1716: mol_type = other DNA
atgaagtgggtgaccttcatcagcctgctgttcctgttctccagcgcctactcctccagctacgtgaggcctctctccgtggctctgggcgaaacagctcgtatcagctgcggtcgtcaagctctgggatctcgtgctgtgcagtggtaccagcaccggcccggtcaagctcccattttactgatctacaacaaccaagatcggccctccggcatccccgaaaggtttagcggcacccccgatatcaacttcggcacaagggccactttaaccattagcggagtggaggccggcgacgaggccgactactactgccacatgtgggactcccggtccggcttttcttggagctttggcggcgctactcgtctgacagtgctgggcggaggcggctccggaggcggcggcagcggaggaggcggatcccaagttcagctgcaagaatccggacccggtttagtgaagcccagcgagactttaagcgtgacttgtagcgtgagcggcgacagcatgaacaactactactggacttggattcgtcagagccccggtaagggtttagagtggatcggctacatctccgaccgggagtccgccacctacaacccctctttaaactcccgggtggtgatctctcgtgacacctccaagaaccagctgtctttaaagctgaactccgtgacccccgctgacaccgccgtgtactactgcgctaccgctaggcggggccagaggatctacggcgtggtgagcttcggcgagttcttctactactacagcatggacgtgtggggcaaaggcaccaccgtgaccgtgtcctccatcacgtgtcctcctcctatgtccgtggaacacgcagacatctgggtcaagagctacagcttgtactccagggagcggtacatttgtaactctggtttcaagcgtaaagccggcacgtccagcctgacggagtgcgtgttgaacaaggccacgaatgtcgcccactggacaacccccagtctcaaatgcattagagagccgaaatcttgtgacaaaactcacacatgcccaccgtgcccagcacctgaactcctggggggaccgtcagtcttcctcttccccccaaaacccaaggacaccctcatgatctcccggacccctgaggtcacatgcgtggtggtggacgtgagccacgaagaccctgaggtcaagttcaactggtacgtggacggcgtggaggtgcataatgccaagacaaagccgcgggaggagcagtacaacagcacgtaccgtgtggtcagcgtcctcaccgtcctgcaccaggactggctgaatggcaaggagtacaagtgcaaggtctccaacaaagccctcccagcccccatcgagaaaaccatctccaaagccaaagggcagccccgagaaccacaggtgtacaccctgcccccatcccgggatgagctgaccaagaaccaggtcagcctgacctgcctggtcaaaggcttctatcccagcgacatcgccgtggagtgggagagcaatgggcagccggagaacaactacaagaccacgcctcccgtgctggactccgacggctccttcttcctctacagcaagctcaccgtggacaagagcaggtggcagcaggggaacgtcttctcatgctccgtgatgcatgaggctctgcacaaccactacacgcagaagagcctctccctgtctcctggtaaataa

SEQ ID NO: 51 - protein, 554 aa, synthetic construct
  REGION 1..554: note = Description of Artificial Sequence: Synthetic polypeptide
MKWVTFISLLFLFSSAYSYIHVTQSPSSLSVSIGDRVTINCQTSQGVGSDLHWYQHKPGRAPKLLIHHTSSVEDGVPSRFSGSGFHTSFNLTISDLQADDIATYYCQVLQFFGRGSRLHIKGGGGSGGGGSGGGGSRAHLVQSGTAMKKPGASVRVSCQTSGYTFTAHILFWFRQAPGRGLEWVGWIKPQYGAVNFGGGFRDRVTLTRDVYREIAYMDIRGLKPDDTAVYYCARDRSYGDSSWALDAWGQGTTVWSAITCPPPMSVEHADIWVKSYSLYSRERYICNSGFKRKAGTSSLTECVLNKATNVAHWTTPSLKCIREPKSCDKTHTCPPCPAPELLGGPSVFLFPPKPKDTLMISRTPEVTCVVVDVSHEDPEVKFNWYVDGVEVHNAKTKPREEQYNSTYRVVSVLTVLHQDWLNGKEYKCKVSNKALPAPIEKTISKAKGQPREPQVYTLPPSRDELTKNQVSLTCLVKGFYPSDIAVEWESNGQPENNYKTTPPVLDSDGSFFLYSKLTVDKSRWQQGNVFSCSVMHEALHNHYTQKSLSLSPGK

SEQ ID NO: 52 - protein, 559 aa, synthetic construct
  REGION 1..559: note = Description of Artificial Sequence: Synthetic polypeptide
MKWVTFISLLFLFSSAYSVVMTQSPSTLSASVGDTITITCRASQSIETWLAWYQQKPGKAPKLLIYKASTLKTGVPSRFSGSGSGTEFTLTISGLQFDDFATYHCQHYAGYSATFGQGTRVEIKGGGGSGGGGSGGGGSEVQLVESGGGLVKAGGSLILSCGVSNFRISAHTMNWVRRVPGGGLEWVASISTSSTYRDYADAVKGRFTVSRDDLEDFVYLQMHKMRVEDTAIYYCARKGSDRLSDNDPFDAWGPGTVVTVSPITCPPPMSVEHADIWVKSYSLYSRERYICNSGFKRKAGTSSLTECVLNKATNVAHWTTPSLKCIREPKSCDKTHTCPPCPAPELLGGPSVFLFPPKPKDTLMISRTPEVTCVVVDVSHEDPEVKFNWYVDGVEVHNAKTKPREEQYNSTYRVVSVLTVLHQDWLNGKEYKCKVSNKALPAPIEKTISKAKGQPREPQVYTLPPSRDELTKNQVSLTCLVKGFYPSDIAVEWESNGQPENNYKTTPPVLDSDGSFFLYSKLTVDKSRWQQGNVFSCSVMHEALHNHYTQKSLSLSPGK

SEQ ID NO: 53 - protein, 557 aa, synthetic construct
  REGION 1..557: note = Description of Artificial Sequence: Synthetic polypeptide
MKWVTFISLLFLFSSAYSSSLTQSPGTLSLSPGETAIISCRTSQYGSLAWYQQRPGQAPRLVIYSGSTRAAGIPDRFSGSRWGPDYNLTISNLESGDFGVYYCQQYEFFGQGTKVQVDIKGGGGSGGGGSGGGGSQVRLSQSGGQMKKPGDSMRISCRASGYEFINCPINWIRLAPGKRPEWMGWMKPRHGAVSYARQLQGRVTMTRDMYSETAFLELRSLTSDDTAVYFCTRGKYCTARDYYNWDFEHWGQGTPVTVSSITCPPPMSVEHADIWVKSYSLYSRERYICNSGFKRKAGTSSLTECVLNKATNVAHWTTPSLKCIREPKSCDKTHTCPPCPAPELLGGPSVFLFPPKPKDTLMISRTPEVTCVVVDVSHEDPEVKFNWYVDGVEVHNAKTKPREEQYNSTYRVVSVLTVLHQDWLNGKEYKCKVSNKALPAPIEKTISKAKGQPREPQVYTLPPSRDELTKNQVSLTCLVKGFYPSDIAVEWESNGQPENNYKTTPPVLDSDGSFFLYSKLTVDKSRWQQGNVFSCSVMHEALHNHYTQKSLSLSPGK

SEQ ID NO: 54 - protein, 571 aa, synthetic construct
  REGION 1..571: note = Description of Artificial Sequence: Synthetic polypeptide
MKWVTFISLLFLFSSAYSSSYVRPLSVALGETARISCGRQALGSRAVQWYQHRPGQAPILLIYNNQDRPSGIPERFSGTPDINFGTRATLTISGVEAGDEADYYCHMWDSRSGFSWSFGGATRLTVLGGGGSGGGGSGGGGSQVQLQESGPGLVKPSETLSVTCSVSGDSMNNYYWTWIRQSPGKGLEWIGYISDRESATYNPSLNSRVVISRDTSKNQLSLKLNSVTPADTAVYYCATARRGQRIYGVVSFGEFFYYYSMDVWGKGTTVTVSSITCPPPMSVEHADIWVKSYSLYSRERYICNSGFKRKAGTSSLTECVLNKATNVAHWTTPSLKCIREPKSCDKTHTCPPCPAPELLGGPSVFLFPPKPKDTLMISRTPEVTCVVVDVSHEDPEVKFNWYVDGVEVHNAKTKPREEQYNSTYRVVSVLTVLHQDWLNGKEYKCKVSNKALPAPIEKTISKAKGQPREPQVYTLPPSRDELTKNQVSLTCLVKGFYPSDIAVEWESNGQPENNYKTTPPVLDSDGSFFLYSKLTVDKSRWQQGNVFSCSVMHEALHNHYTQKSLSLSPGK

SEQ ID NO: 55 - protein, 6 aa, synthetic construct
  REGION 1..6: note = Description of Artificial Sequence: Synthetic peptide
PELLGG

SEQ ID NO: 56 - protein, 6 aa, synthetic construct
  REGION 1..6: note = Description of Artificial Sequence: Synthetic peptide
PEAAGG

SEQ ID NO: 57 - protein, 5 aa, synthetic construct
  REGION 1..5: note = Description of Artificial Sequence: Synthetic peptide
KCKSL

SEQ ID NO: 58 - protein, 5 aa, synthetic construct
  REGION 1..5: note = Description of Artificial Sequence: Synthetic peptide
KCASL